European Patent Application EP 4 600 360 A1, published August 13, 2025. Title: METHOD FOR PRODUCING POLYHYDROXYALKANOATE COPOLYMER MIXTURE AND TRANSFORMED MICROORGANISM. Applicant: KANEKA CORPORATION. Application JP. The sequence listing filed with the application follows.

SEQUENCE LISTING (52 sequences)

SEQ ID NO: 1 - protein, 594 aa, Aeromonas sp.
MSQPSYGPLFEALAHYNDKLLAMAKAQTERTAQALLQTNLDDLGQVLEQGSQQPWQLIQAQMNWWQDQLKLMQHTLLKSAGQPSEPVITPERSDRRFKAEAWSEQPIYDYLKQSYLLTARHLLASVDALEGVPQKSRERLRFFTRQYVNAMAPSNFLATNPELLKLTLESDGQNLVRGLALLAEDLERSADQLNIRLTDESAFELGRDLALTPGRVVQRTELYELIQYSPTTETVGKTPVLIVPPFINKYYIMDMRPQNSLVAWLVAQGQTVFMISWRNPGVAQAQIDLDDYVVDGVIAALDGVEAATGEREVHGIGYCIGGTALSLAMGWLAARRQKQRVRTATLFTTLLDFSQPGELGIFIHEPIIAALEAQNEAKGIMDGRQLAVSFSLLRENSLYWNYYIDSYLKGQSPVAFDLLHWNSDSTNVAGKTHNSLLRRLYLENQLVKGELKIRNTRIDLGKVKTPVLLVSAVDDHIALWQGTWQGMKLFGGEQRFLLAESGHIAGIINPPAANKYGFWHNGAEAESPESWLAGATHQGGSWWPEMMGFIQNRDEGSEPVPARVPEEGLAPAPGHYVKVRLNPVFACPTEEDAA

SEQ ID NO: 2 - protein, 594 aa, Aeromonas sp.
MSQPSYGPLFEALAHYNDKLLAMAKAQTERTAQALLQTNLDDLGQVLEQGSQQPWQLIQAQMNWWQDQLKLMQHTLLKSAGQPSEPVITPERSDRRFKAEAWSEQPIYDYLKQSYLLTARHLLASVDALEGVPQKSRERLRFFTRQYVSAMAPSNFLATNPELLKLTLESGGQNLVRGLALLAEDLERSADQLNIRLTDESAFELGRDLALTPGRVVQRTELYELIQYSPTTETVGKTPVLIVPPFINKYYIMDMRPQNSLVAWLVAQGQTVFMISWRNPGVAQAQIDLDDYVVDGVIAALDGVEAATGEREVHGIGYCIGGTALSLAMGWLAARRQKQRVRTATLFTTLLDFSQPGELGIFIHEPIIAALEAQNEAKGIMDGRQLAVSFSLLRENSLYWNYYIDSYLKGQSPVAFDLLHWNSDSTNVAGKTHNSLLRRLYLENQLVKGELKIRNTRIDLGKVKTPVLLVSAVDDHIALWQGTWQGMKLFGGEQRFLLAESGHIAGIINPPAANKYGFWHNGAEAESPESWLAGATHQGGSWWPEMMGFIQNRDEGSEPVPARVPEEGLAPAPGHYVKVRLNPVFACPTEEDAA

SEQ ID NO: 3 - protein, 594 aa, Aeromonas sp.
MSQPSYGPLFEALAHYNDKLLAMAKAQTERTAQALLQTNLDDLGQVLEQGSQQPWQLIQAQMNWWQDQLKLMQHTLLKSAGQPSEPVITPERSDRRFKAEAWSEQPIYDYLKQSYLLTARHLLASVDALEGVPQKSRERLRFFTRQYVSAMAPSNFLATNPELLKLTLESGGQNLVRGLALLAEDLERSADQLNIRLTDESAFELGRDLALTPGRVVQRTELYELIQYSPTTETVGKTPVLIVPPFINKYYIMDMRPQNSLVAWLVAQGQTVFMISWRNPGVAQAQIDLDDYVVDGVIAALDGVEAATGEREVHGIGYCIGGTALSLAMGWLAARRQKQRVRTATLFTTLLDFSQPGELGIFIHEPIIAALEAQNEAKGIMDGRQLAVGFSLLRENSLYWNYYIDSYLKGQSPVAFDLLHWNSDSTNVAGKTHNSLLRRLYLENQLVKGELKIRNTRIDLGKVKTPVLLVSAVDDHIALWQGTWQGMKLFGGEQRFLLAESGHIAGIINPPAANKYGFWHNGAEAESPESWLAGATHQGGSWWPEMMGFIQNRDEGSEPVPARVPEEGLAPAPGHYVKVRLNPVFACPTEEDAA

SEQ ID NO: 4 - protein, 594 aa, Aeromonas sp.
MSQPSYGPLFEALAHYNDKLLAMAKAQTERTAQALLQTNLDDLGQVLEQGSQQPWQLIQAQMNWWQDQLKLMQHTLLKSAGQPSEPVITPERSDRRFKAEAWSEQPIYDYLKQSYLLTARHLLASVDALEGVPQKSRERLRFFTRQYVSAMAPSNFLATNPELLKLTLESGGQNLVRGLALLAEDLERSADQLNIRLTDESAFELGRDLALTPGRVVQRTELYELIQYSPTTETVGKTPVLIVPPFINKYYIMDMRPQNSLVAWLVAQGQTVFMISWRNPGVAQAQIDLDDYVVDGVIAALDGVEAATGEREVHGIGYCIGGTALSLAMGWLAARRQKQRVRTATLFTTLLDFSQPGELGIFIHEPIIAALEAQNEAKGIMDGRQLAVPFSLLRENSLYWNYYIDSYLKGQSPVAFDLLHWNSDSTNVAGKTHNSLLRRLYLENQLVKGELKIRNTRIDLGKVKTPVLLVSAVDDHIALWQGTWQGMKLFGGEQRFLLAESGHIAGIINPPAANKYGFWHNGAEAESPESWLAGATHQGGSWWPEMMGFIQNRDEGSEPVPARVPEEGLAPAPGHYVKVRLNPVFACPTEEDAA

SEQ ID NO: 5 - protein, 594 aa, Aeromonas sp.
MSQPSYGPLFEALAHYNDKLLAMAKAQTERTAQALLQTNLDDLGQVLEQGSQQPWQLIQAQMNWWQDQLKLMQHTLLKSAGQPSEPVITPERSDRRFKAEAWSEQPIYDYLKQSYLLTARHLLASVDALEGVPQKSRERLRFFTRQYVSAMAPSNFLATNPELLKLTLESGGQNLVRGLALLAEDLERSADQLNIRLTDESAFELGRDLALTPGRVVQRTELYELIQYSPTTETVGKTPVLIVPPFINKYYIMDMRPQNSLVAWLVAQGQTVFMISWRNPGVAQAQIDLDDYVVDGVIAALDGVEAATGEREVHGIGYCIGGTALSLAMGWLAARRQKQRVRTATLFTTLLDFSQPGELGIFIHEPIIAALEAQNEAKGIMDGRQLAVCFSLLRENSLYWNYYIDSYLKGQSPVAFDLLHWNSDSTNVAGKTHNSLLRRLYLENQLVKGELKIRNTRIDLGKVKTPVLLVSAVDDHIALWQGTWQGMKLFGGEQRFLLAESGHIAGIINPPAANKYGFWHNGAEAESPESWLAGATHQGGSWWPEMMGFIQNRDEGSEPVPARVPEEGLAPAPGHYVKVRLNPVFACPTEEDAA

SEQ ID NO: 6 - protein, 594 aa, Aeromonas sp.
MSQPSYGPLFEALAHYNDKLLAMAKAQTERTAQALLQTNLDDLGQVLEQGSQQPWQLIQAQMNWWQDQLKLMQHTLLKSAGQPSEPVITPERSDRRFKAEAWSEQPIYDYLKQSYLLTARHLLASVDALEGVPQKSRERLRFFTRQYVSAMAPSNFLATNPELLKLTLESGGQNLVRGLALLAEDLERSADQLNIRLTDESAFELGRDLALTPGRVVQRTELYELIQYSPTTETVGKTPVLIVPPFINKYYIMDMRPQNSLVAWLVAQGQTVFMISWRNPGVAQAQIDLDDYVVDGVIAALDGVEAATGEREVHGIGYCIGGTALSLAMGWLAARRQKQRVRTATLFTTLLDFSQPGELGIFIHEPIIAALEAQNEAKGIMDGRQLAVIFSLLRENSLYWNYYIDSYLKGQSPVAFDLLHWNSDSTNVAGKTHNSLLRRLYLENQLVKGELKIRNTRIDLGKVKTPVLLVSAVDDHIALWQGTWQGMKLFGGEQRFLLAESGHIAGIINPPAANKYGFWHNGAEAESPESWLAGATHQGGSWWPEMMGFIQNRDEGSEPVPARVPEEGLAPAPGHYVKVRLNPVFACPTEEDAA

SEQ ID NO: 7 - protein, 594 aa, Aeromonas sp.
MSQPSYGPLFEALAHYNDKLLAMAKAQTERTAQALLQTNLDDLGQVLEQGSQQPWQLIQAQMNWWQDQLKLMQHTLLKSAGQPSEPVITPERSDRRFKAEAWSEQPIYDYLKQSYLLTARHLLASVDALEGVPQKSRERLRFFTRQYVSAMAPSNFLATNPELLKLTLESGGQNLVRGLALLAEDLERSADQLNIRLTDESAFELGRDLALTPGRVVQRTELYELIQYSPTTETVGKTPVLIVPPFINKYYIMDMRPQNSLVAWLVAQGQTVFMISWRNPGVAQAQIDLDDYVVDGVIAALDGVEAATGEREVHGIGYCIGGTALSLAMGWLAARRQKQRVRTATLFTTLLDFSQPGELGIFIHEPIIAALEAQNEAKGIMDGRQLAVVFSLLRENSLYWNYYIDSYLKGQSPVAFDLLHWNSDSTNVAGKTHNSLLRRLYLENQLVKGELKIRNTRIDLGKVKTPVLLVSAVDDHIALWQGTWQGMKLFGGEQRFLLAESGHIAGIINPPAANKYGFWHNGAEAESPESWLAGATHQGGSWWPEMMGFIQNRDEGSEPVPARVPEEGLAPAPGHYVKVRLNPVFACPTEEDAA

SEQ ID NO: 8 - protein, 594 aa, Aeromonas sp.
MSQPSYGPLFEALAHYNDKLLAMAKAQTERTAQALLQTNLDDLGQVLEQGSQQPWQLIQAQMNWWQDQLKLMQHTLLKSAGQPSEPVITPERSDRRFKAEAWSEQPIYDYLKQSYLLTARHLLASVDALEGVPQKSRERLRFFTRQYVSAMAPSNFLATNPELLKLTLESGGQNLVRGLALLAEDLERSADQLNIRLTDESAFELGRDLALTPGRVVQRTELYELIQYSPTTETVGKTPVLIVPPFINKYYIMDMRPQNSLVAWLVAQGQTVFMISWRNPGVAQAQIDLDDYVVDGVIAALDGVEAATGEREVHGIGYCIGGTALSLAMGWLAARRQKQRVRTATLFTTLLDFSQPGELGIFIHEPIIAALEAQNEAKGIMDGRQLAVTFSLLRENSLYWNYYIDSYLKGQSPVAFDLLHWNSDSTNVAGKTHNSLLRRLYLENQLVKGELKIRNTRIDLGKVKTPVLLVSAVDDHIALWQGTWQGMKLFGGEQRFLLAESGHIAGIINPPAANKYGFWHNGAEAESPESWLAGATHQGGSWWPEMMGFIQNRDEGSEPVPARVPEEGLAPAPGHYVKVRLNPVFACPTEEDAA

SEQ ID NO: 9 - protein, 551 aa, unidentified
MASKDSFGKTGDLWSSMFNWMSGTMTAAAQIQQANMRAFAQSMELATSAYARMWGQPVEQVVPADRRFKDEAWTENMAADLLKQSYLITSQWLMEIADGWQAIDPDLHERTRFWTQQLVDATSPANFAMTNPVVMQEIARTGGMNLIQGAQNLLKDAQSGRLTQVPEDAFEVGKDLAITPGKVVYRNRLIELIQYTPATETVHEIPILVVPPWINKYYVMDMQPENSLFKYLVDAGFTLFTISWKNPDETVLDLEWDDYLDLGTLEALRMVKEIMGVEQVNLVGYCLGGIISQVTLAYLAATGDDAQINSATYFTTHQDFSDAGEISVFISRLDVMFLEWLMKISGGYLDGRNLAATFNMLRANDLLWNYVVHNYLLGQEPASFDLLYWNNDGTRVPGKVHSFLLREFFLDNKLKEPEGIQVKGVGIDLGKITTPTYVVTADRDHIVPWRGAFLVRQLQSGPVRFILSGGGHIAGVISPPTKNRGFWINEEEKDDADAWLAGATKHDGSWWVDWIPWLEERSGRRVKPPTAAGSDEFKPLMDAPGTYVLEK

SEQ ID NO: 10 - protein, 585 aa, synthetic construct
MSQPSYGPLFEALAHYNDKLLAMAKAQTERTAQALLQTNLDDLGQVLEQGSQQPWQLIQAQMNWWQDQLKLMQHTLLKSAGQPSEPVITPERSDRRFKAEAWSEQPIYDYLKQSYLLTARHLLASVDALEGVPQKSRERLRFFTRQYVSAMAPANFLATNPEAQRLLIESGGESLRAGVRNMMEDLTRGKISQTDESAFEVGRNVAVTEGAVVFENEYFQLLQYKPLTDKVHARPLLMVPPCINKYYILDLQPESSLVRHVVEQGHTVFLVSWRNPDASMAGSTWDDYIEHAAIRAIEVARDISGQDKINVLGFCVGGTIVSTALAVLAARGEHPAASVTLLTTLLDFADTGILDVFVDEGHVQLREATLGGGAGAPCALLRGLELANTFSFLRPNDLVWNYVVDNYLKGNTPVPFDLLFWNGDATNLPGPWYCWYLRHTYLQNELKVPGKLTVCGVPVDLASIDVPTYIYGSREDHIVPWTAAYASTALLANKLRFVLGASGHIAGVINPPAKNKRSHWTNDALPESPQQWLAGAIEHHGSWWPDWTAWLAGQAGAKRAAPANYGNARYRAIEPAPGRYVKAKA

SEQ ID NO: 11 - protein, 585 aa, synthetic construct
MSQPSYGPLFEALAHYNDKLLAMAKAQTERTAQALLQTNLDDLGQVLEQGSQQPWQLIQAQMNWWQDQLKLMQHTLLKSAGQPSEPVITPERSDRRFKAEAWSEQPIYDYLKQSYLLTARHLLASVDALEGVPQKSRERLRFFTRQYVSAMAPANFLATNPEAQRLLIESGGESLRAGVRNMMEDLTRGKISQTDESAFEVGRNVAVTEGAVVFENEYFQLLQYKPLTDKVHARPLLMVPPCINKYYILDLQPESSLVRHVVEQGHTVFLVSWRNPDASMAGSTWDDYIEHAAIRAIEVARDISGQDKINVLGFCVGGTIVSTALAVLAARGEHPAASVTLLTTLLDFADTGILDVFVDEGHVQLREATLGGGAGAPCALLRGLELANTFSFLRPNDLVWNYVVDNYLKGNTPVPFDLLFWNGDATNLPGPWYCWYLRHTYLQNELKVPGKLTVCGVPVDLASIDVPTYIYGSREDHIVPWTAAYASTALLANKLRFVLGASGHIMGVINPPAKNKRSHWTNDALPESPQQWLAGAIEHHGSWWPDWTAWLAGQAGAKRAAPANYGNARYRAIEPAPGRYVKAKA

SEQ ID NO: 12 - protein, 567 aa, Chromobacterium sp.
MQQFVNSLSLGQDQSDAPHPLTGAWSQLMSQTNQLLQLQSSLYQQQLGLWTQFLGQTAGNDASAPSAKPSDRRFASPEWDEHPFYSFLKQSYLQTSKWMMELVDKTQIDESAKDKLSFATRQYLDAMAPSNFMLTNPDVVKRAIETQGESLVEGMKNMMEDIQKGHISMSDESKFQIGKNLVVTPGEVVFRNELIELIQYTPTTEKVHEKPLLFVPPCINKYYLMDLQPDNSMVRHFVGQGYRVFLVSWRSAVPEMKNFTWETYIEKGVFAAAEAVQKITKQPTMNALGFCVGGVILTTALCVAQAKGLKYFDSATFMTSLIDHAEPGEISFFIDEALVASREAKMAAGGIISGKEIGRTFASLRANDLVWNYVVNNYLLGKTPAPFDLLYWNNDAVDLPLPMHTFMLRQFYINNALITPGAITLCGVPIDISKIDIPVYMFAAREDHIVLWSSAYSGLKYLSGTPSRRFVLGASGHIWGSINPVTKDKRNYWTNEQLPVNPEEWLEGAQSHPGSWWKDWDAWLAPQSGKQVPAPKMLGSKEFPPLQPAPGSYVLAKAMPPVAAALN

SEQ ID NO: 13 - protein, 567 aa, Chromobacterium sp.
MQQFVNSLSLGQDQSDAPHPLTGAWSQLMSQTNQLLQLQSSLYQQQLGLWTQFLGQTAGNDASAPSAKPSDRRFASPEWDEHPFYSFLKQSYLQTSKWMMELVDKTQIDESAKDKLSFATRQYLDAMAPSNFMLTNPDVVKRAIETQGESLVEGMKNMMEDIQKGHISMSDESKFQIGKNLVVTPGEVVFRNELIELIQYTPTTEKVHEKPLLFVPPCINKYYLMDLQPDNSMVRHFVGQGYRVFLVSWRSAVPEMKNFTWETYIEKGVFAAAEAVQKITKQPTMNALGFCVGGVILTTALCVAQAKGLKYFDSATFMTSLIDHAEPGEISFFIDEALVASREAKMAAGGIISGKEIGRTFASLRANDLVWNYVVNNYLLGKTPAPFDLLYWNNDAVDLPLPMHTFMLRQFYINNALITPGAITLCGVPIDISKIDIPVYMFAAREDHIVLWSSAYSGLKYLSGTPSRRFVLGASGHIMGSINPVTKDKRNYWTNEQLPVNPEEWLEGAQSHPGSWWKDWDAWLAPQSGKQVPAPKMLGSKEFPPLQPAPGSYVLAKAMPPVAAALN

SEQ ID NO: 14 - protein, 134 aa, Aeromonas caviae
MSAQSLEVGQKARLSKRFGAAEVAAFAALSEDFNPLHLDPAFAATTAFERPIVHGMLLASLFSGLLGQQLPGKGSIYLGQSLSFKLPVFVGDEVTAEVEVTALREDKPIATLTTRIFTQGGALAVTGEAVVKLP

SEQ ID NO: 15 - protein, 158 aa, Cupriavidus necator
MRTIASLEELEGLQGQEVAVSDWIEVTQQQVNQFADATGDHQWIHIDVERAKKESPYGGPIAHGFLTLSLLPKFMHNALHMPSKIGVNYGLNRVRFTAPVPVGSKLRARIKLLKVERLDPLPKSPELVGAQSTWEVTVEREGSDRPVCVAESITRRYG

SEQ ID NO: 16 - protein, 151 aa, Cupriavidus necator
MKTYENIADLQPLVGEVIGTSEWLALDQARINTFADATGDHQWIHVDVERAKNGPFGAPIAHGFLTLSLLPAFTHSAYRIRNSSTGVNYGLDKVRFPAPVPVDSLLRAQFKLMSYEALENGGAQFKVEMMVERQGGSKPVCIAESILRRFP

SEQ ID NO: 17 - protein, 901 aa, Yarrowia lipolytica
MSGELRYDGKVVIVTGAGGGLGKAYALFYGSRGASVVVNDLGGDFKGDGAQAGSGKRVADVVVDEIVSKGGKAVANYDSVENGDKIVETAVKAFGSVHIVINNAGILRDISFKKMTDKDWDLVYKVHVFGAYKVTRAAWPYFRKQKYGRVISTSSAAGLYGNFGQTNYSAAKLALVGFGETLAKEGAKYNITSNVIAPLAASRMTETVMPEDILKLLKPEYVVPLVGYLTHDSVTESYGIYEVGAGYMAKIRWERGNGAVFKGDDTFTPSAILKRWDEVTSFESPTYPNGPADFFKYAEESVKRPENPQGPTVSFKDQVVIVTGAGAGIGRAYSHLLAKLGAKVVVNDFGNPQKVVDEIKALGGIAVADKNNVIHGEKVVQTAIDAFGAVHAVVNNAGILRDKSFANMDDEMWQLIFDVHLNGTYSVTKAAWPHFLKQKYGRVINTTSTSGIYGNFGQANYSAAKAGILGFSRALAREGEKYNILVNTIAPNAGTAMTASVFTEEMLELFKPDFIAPITVLLASDQAPVTGDLFETGSAWIGQTRWQRAGGKAFNTKKGVTPEMVRDSWAKIVDFDDGNSTHPTTPSESTTQILENIFNVPDEEVEETALVAGPGGPGILNKEGEPFDYTYTYRDLILYNLGLGAKANELKYVFEGDDDFQTVPTFGVIPYMGGLITTNYGDFVPNFNPMMLLHGEQYLEIRQWPIPTNATLENKAKVIDVVDKGKAALLVTATTTTNKETGEEVFYNESSLFIRGSGGFGGKSTGTDRGAATAANKPPARAPDFVKEIKIQEDQAAIYRLSGDYNPLHIDPAFAAVGNFDRPILHGLCSFGVSGKALYDQFGPFKNAKVRFAGHVFPGETLKVEGWKEGNKVIFQTKVVERGTTAISNAAIELFPKDAKL

SEQ ID NO: 18 - protein, 598 aa, Drosophila melanogaster
MSSSDGKLRYDGRVAVVTGAGAGLGREYALLFAERGAKVVVNDLGGTHSGDGASQRAADIVVDEIRKAGGEAVADYNSVIDGAKVIETAIKAFGRVDILVNNAGILRDRSLVKTSEQDWNLVNDVHLKGSFKCTQAAFPYMKKQNYGRIIMTSSNSGIYGNFGQVNYTAAKMGLIGLANTVAIEGARNNVLCNVIVPTAASRMTEGILPDILFNELKPKLIAPVVAYLCHESCEDNGSYIESAAGWATKLHMVRGKGAVLRPSLDDPVTIEYVKDVWSNVTDMSKAKHLGAIAEASGTLLEVLEKLKEGGGDAIEDAFEFNSKELITYALGIGASVKNAKDMRFLYENDADFAAIPTFFVLPGLLLQMSTDKLLSKALPNSQVDFSNILHGEQYLEIVDDLPTSGTLLTNGKVFDVMDKGSGAVVVTNSESFDESGRLLVRNQSTTFIVGAGKFGGKKDPIAGVVPLQPAPNRQPDATVQYTTSEDQAALYRLSGDKNPLHIDPQMALLAGFKTPILHGLCTLGFSVRAVLAQFADNNPALFKAVKVRFSGPVIPGQTLRVDLWKQGTRINFRTVVVETGKEVISGAYVDLKSSQAKL

SEQ ID NO: 19 - protein, 394 aa, Cupriavidus necator
MTREVVVVSGVRTAIGTFGGSLKDVAPAELGALVVREALARAQVSGDDVGHVVFGNVIQTEPRDMYLGRVAAVNGGVTINAPALTVNRLCGSGLQAIVSAAQTILLGDTDVAIGGGAESMSRAPYLAPAARWGARMGDAGLVDMMLGALHDPFHRIHMGVTAENVAKEYDISRAQQDEAALESHRRASAAIKAGYFKDQIVPVVSKGRKGDVTFDTDEHVRHDATIDDMTKLRPVFVKENGTVTAGNASGLNDAAAAVVMMERAEAERRGLKPLARLVSYGHAGVDPKAMGIGPVPATKIALERAGLQVSDLDVIEANEAFAAQACAVTKALGLDPAKVNPNGSGISLGHPIGATGALITVKALHELNRVQGRYALVTMCIGGGQGIAAIFERI

SEQ ID NO: 20 - protein, 392 aa, Cupriavidus necator
MNEAVIVSTARTPLAKSWKGAFNMTHGATLGGHAVQHAIARAKIEAAEVEDVLMGCANPEGATGANIARQIALRAGCPVTVPGATVNRFCSSGLQTIAMAAQRVIADEGDIFVAGGVESISCVQQEMNRHMVQESWLLKNKPEIYWNMLQTAENVAKRYNISKERQDEYGVRSQQRAAAGQEAGKFKDEIVPMTVLAGVADKSTGQLVTKEVTVSADEGIRADTTLEGVSKIRSAVPGGVITAGNASQFSDGASAAVVMNARVAEARGLQPLGVFRGFAVAGCEPDEMGIGPVFAVPKLLKKAGLKVDDIGLWELNEAFAVQVLYCADTLGIPMDRLNVNGGAIAVGHPYGVSGARLVGHALIEGKRRGVKYVVVTMCIGGGQGAAGLFEVL

SEQ ID NO: 21 - DNA, 29 bp, Escherichia coli
  source 1..29: mol_type = other DNA
tttacacttatgcttccggctcgtatgtt

SEQ ID NO: 22 - DNA, 31 bp, Escherichia coli
  source 1..31: mol_type = other DNA
tttacacctttatgcttccggctcgtatgtt

SEQ ID NO: 23 - DNA, 1056 bp, synthetic construct
  source 1..1056: mol_type = other DNA
gcgcgcatttaaatctgccaccacgttgtgctcggtgatcgccatcatcagcgccacgtagagccagccaatggccacgatgtacatcaaaaattcatccttctcgcctatgctctggggcctcggcagatgcgagcgctgcataccgtccggtaggtcgggaagcgtgcagtgccgaggcggattcccgcattgacagcgcgtgcgttgcaaggcaacaatggactcaaatgtctcggaatcgctgacgattcccaggtttctccggcaagcatagcgcatggcgtctccatgcgagaatgtcgcgcttgccggataaaaggggagccgctatcggaatggacgcaagccacggccgcagcaggtgcggtcgagggcttccagccagttccagggcagatgtgccggcagaccctcccgctttgggggaggcgcaagccgggtccattcggatagcatctccccatgcaaagtgccggccagggcaatgcccggagccggttcgaatagtgacggcagagagacaatcaaatccgcttgcatgagtgccggcgtgcgtcatgcacggcgccggcaggcctgcaggttccctcccgtttccattgaaaggactacacaatgactgacgttgtcatcgtatccgccgcccgcaccgcggtcggcaagtttggcggctcgctggccaagatcccggcaccggaactgggtgccgtggtcatcaaggccgcgctggagcgcgccggcgtcaagccggagcaggtgagcgaagtcatcatgggccaggtgctgaccgccggttcgggccagaaccccgcacgccaggccgcgatcaaggccggcctgccggcgatggtgccggccatgaccatcaacaaggtgtgcggctcgggcctgaaggccgtgatgctggccgccaacgcgatcatggcgggcgacgccgagatcgtggtggccggcggccaggaaaacatgagcgccgccccgcacgtgctgccgggctcgcgcgatggtttccgcatgggcgatgccaagctggtcgacaatttaaatgcgcgc

SEQ ID NO: 24 - DNA, 2740 bp, synthetic construct
  source 1..2740: mol_type = other DNA
atccatttaaatcaggcacttgaagcacgcgacggcaagcggcttgcggccatcctgcgccagcacctcctggacaagcgcgacgcggtgctgctgatccaggcaggcgatgccgttggcacgccccaggcataggacgctggcgccaccctcaccccaagaatccgaatagccccatcagcattctttgccccgctgtcaccacggtgacaaccccggttcttactctgcgagcgcattgcggcaaacgcaatccgccatgcggcacctgccgcagcgcacaacaacgcagatgaacaggggaatcaaagatggcagggaaccttgcaccggacaggctggcggggatgtcgcgcggccgtcaattctgcttctggcgtcaggcagccatcggaagctgtggtatggctgtgcaggtcgtaaatcactgcataattcgtgtcgctcaaggcgcactcccgttctggataatgttttttgcgccgacatcataacggttctggcaaatattctgaaatgagctgttgacaattaatcatcgaactagttaactagtacgcaagttcacagcggataacaatttcacacaggaaacaattgcacgtgcagagagacaatcaaatcatgcagcagtttgtcaattccctgtcgctcggccaggaccagtccgatgccccccatccgctgaccggcgcctggtcgcagctgatgagccagaccaatcagctcttgcagctgcaatccagcctctaccaacagcaattgggcttgtggacgcaattcctcggccaaaccgccggcaacgacgcttccgcgccgtcggccaagccgagcgaccgccgcttcgcctcgccggagtgggatgagcatccgttctacagcttcctcaagcagagctatctgcaaacctccaagtggatgatggagctggtggacaagacccagatcgacgaaagcgctaaggacaagctgtccttcgccactcgccagtacctggatgccatggcgcccagcaacttcatgctgaccaaccccgacgtggtcaaacgcgccatcgaaacccagggcgaaagcctggtggaaggcatgaagaacatgatggaggacatccagaagggccatatctcgatgtccgacgagagcaagttccaaatcggcaaaaacctggtggtgacgccgggcgaggtggtgttccgcaatgaactgatcgagctgatccagtacacgccgaccaccgaaaaagtccacgaaaagcccttgctgtttgtcccgccgtgcatcaacaagtactacctgatggatctgcagccggacaactccatggtgcgccacttcgtcggccagggttaccgcgttttcctggtcagctggcgttccgccgtgcccgagatgaagaacttcacttgggagacctacatcgagaaaggcgtgttcgccgcggccgaagcggttcagaagatcaccaagcagccgaccatgaacgcgctgggcttctgcgtgggcggcgtgatcctcactaccgcgctgtgcgtggcccaggccaagggtctgaaatacttcgactccgccaccttcatgacgtcgctgatcgaccacgccgaaccgggcgagatctccttcttcatcgacgaggcgctggtagccagccgcgaagccaaaatggcggccggcggcatcatcagcggcaaggaaatcggacgcactttcgccagcctgcgcgccaacgacctggtgtggaactacgtcgtcaacaactacctgctgggcaagaccccggcgccgttcgacctgctgtactggaacaacgacgcggtggacctgccgctgccgatgcacaccttcatgctgcggcagttctacatcaacaacgcgctgatcaccccgggcgccattacgctgtgcggcgtcccgatcgacatctccaagatcgacatcccggtgtatatgttcgccgcgcgcgaagaccacatcgtgctgtggagttccgcctactccggcctgaaatatctgagcggcacgccaagccgccgctttgtcctgggcgcatccggccacatctggggctcgatcaaccccgtcaccaaggataagcgcaactactggaccaacgagcagctgccggtgaatccggaagaatggctggagggcgcgcaaagccatccaggcagctggtggaaggactgggacgcctggctggccccgcaatccggaaaacaggttccggcgcccaagatgctgggcagcaaggagttccccccgctgcagcctgcgccgggcagctatgtgctcgccaaggcgatgcctcccgtcgccgccgccttgaactgacctgccggcctggttcaaccagtcggcagccggaattgatcgatactagtatccggccggagcccgtttcgtcacggaacgggttcctcaccgacccttcccccccgcccgatcccctgcaggagattgacaccatgactttccgaccttccaccctggcgcggccgcactggctcgccgccgtgctgatgtgcgcagcgctcgccgcctgcggcggcgactccggcgacagccccaccggctcgcccaacgcggcaccgatcacgccgggtgccccgggtaccggcggcaaccccggccaggggaatggcagcgaccagcctggcgagacgcccgccgtgaagccgcagctgcgctgcgcaccctgaagccgggcctggcccgtctcccctccagaaacatttaaatccga

SEQ ID NO: 25 - DNA, 2677 bp, synthetic construct
  source 1..2677: mol_type = other DNA
atccatttaaatcccgggggtggatgcacagacccgcgagatctcggccaagctcgactccggcaagcacaccaccaccttcacgcggctctatcacctgccggccgaatggggcaccgtggacggccatcagggtgcgctgatcgattcgccgggcttccaggaattcggcctgtaccacctgagcgagggcatgctggagcgcgccttcccggagttccgcccgctgctgaccgggtgccgcttctacaactgccaccacgtcaacgagcccggctgcggcgtgctggccgcggtcgcctcgggagcgatctccgagcgccgccaccagctctacatgcagttgctgcacgaatccaaccagcagaagccgtggtaaggtaagcgcacctgggttacccggtgcgctgcccaattgcacgtgcagagagacaatcaaatcatgagccaaccatcttatggcccgctgttcgaggccctggcccactacaatgacaagctgctggccatggccaaggcccagacagagcgcaccgcccaggcgctgctgcagaccaatctggacgatctgggccaggtgctggagcagggcagccagcaaccctggcaactgatccaggcccagatgaactggtggcaggatcagctcaagctgatgcagcacaccctgctcaaaagcgcaggccagccgagcgagccggtgatcaccccggagcgcagcgatcgccgcttcaaggccgaggcctggagcgaacaacccatctatgactacctcaagcagtcctacctgctcaccgccaggcacctgctggcctcggtggatgccctggagggcgtcccccagaagagccgggagcggctgcgtttcttcacccgccagtacgtcagcgccatggcccccagcaacttcctggccaccaaccccgagctgctcaagctgaccctggagtccggcggccagaacctggtgcgcgggctggccctcttggccgaggatctggagcgcagcgccgatcagctcaacatccgcctgaccgacgaatccgccttcgagctcgggcgggatctggcgctcaccccgggccgggtggtgcagcgcaccgagctctatgagctgatccagtacagcccgactaccgagacggtgggcaagacacctgtgctgatagtgccccccttcatcaacaagtactacatcatggacatgcggccccagaactccctggtcgcctggctggtcgcccagggccagacggtgttcatgatctcctggcgcaacccgggcgtggcccaggcccaaatcgatctcgacgactacgtggtggacggggtcatcgccgccctggacggggtggaggcggccaccggcgagcgggaggtgcacggcatcggctactgcatcggcggcactgcactgtcgctcgccatgggctggctggcggcgcggcgccagaagcagcgagtgcgcaccgccaccctgttcactaccctgctggacttctcccagccaggggagctcggcatcttcatccacgagcccatcatagcggcgctcgaggcgcaaaatgaggccaagggcatcatggacgggcgccagctggctgtctccttcagcctgctgcgggagaacagcctctactggaactactacatcgacagctacctcaagggccagagcccggtggccttcgatctgctgcactggaacagcgacagcaccaatgtggcgggcaagacccacaacagcctgctgcgccgtctctacctggagaaccagctggtgaagggggagctcaagatccgcaacacccgcatcgatctcggcaaggtgaaaaccccggtactgctggtgtcggccgtggacgatcacatcgccctctggcagggcacctggcagggcatgaagctgtttggcggggagcagcgcttcctcctggcggagtccggccacatcgccggcatcatcaacccgccggccgccaacaagtacggcttctggcacaacggggccgaggccgagagcccggagagctggctggcaggggcgacgcaccagggcggctcctggtggcccgagatgatgggctttatccagaaccgtgacgaagggtcggagcccgtccccgcgcgggtgcccgaggaggggctggcccccgcccccggccactatgtcaaggtgcggctcaaccccgtgtttgcctgcccaacagaggaggacgccgcatgacctgccggcctggttcaaccagtcggcagccgactagtatgaaactgctgctgtccgccacttccctcgtccatgcagcccattgccggaacgtcctgcgggcggccggcatccgggcggaattgcgcaatacctggctggccggcgcgaccggcgagatcccgttccgggagagtgcgccacaggtgtggctggtcgatgacgagatggaagcgcaggcgtgggcggtgctcaatgccgccgccaacccggcgccggggccgagctggcaatgccgccactgcctggaatggcacgaggcccagttcggggcctgctggcgctgcggcgcggcccgcgactagcgcgccgccccctttttgacgctggtcagccgacccagagcgccagcgacagcatcgccagcagcagcatccacagcaccaccgcgcgccatacatttaaatccga

SEQ ID NO: 26 - DNA, 1009 bp, synthetic construct
  source 1..1009: mol_type = other DNA
gcgcgcatttaaatggagttccagaccctgctcgactttatcgccgaagccgaactggaccgcgtcggctgcttcgcctactcgccggtggagggcgccaccgccaatgacctgccgggcgcgctgcccgacgaggtgcgcgaggaacgccgcgcccgcttcatggaagtggccgaagaggtctcggcgcgccgcctgcagcgcaaggtcggccagaccctgcgcgtgctggtggacgaggtcaaccaggatggcggcatcggccgttcgtccgcggatgcgccggaaatcgacggcctcgtctatatcgcgccgccggaacgccacgcccagcgctatcgcgccggcgagttcgtcgacgtgaagatcaccggcgccgatggccacgacctgtggggcgcggtctgaaacgggttgattaggtaaaagtacgctcgttcgatttcgtccgcgtcccgctatactgtgcggtgcaacataacctcatggagacaaagtcggttagccttgcgccttgcttcgctgacgaagaacctctgcgcgctcggcctggccgccgtgctcgcgctggcgggcacggcgcaggcagcgccggcgaccgagctgtcgaccggcccggttaacaccgggccagccggcggcgaaggcctgggcatcaaccaggccattcgcgacggcgaagcccggcgcggcggcacctcgctttccactggcgcgccaaaacccctggcgccgcggccggaatatgcgtcgctgccggtctacgtcggcaaggtcggcgaccagccggtgcggctgcgcctgggccccaagcctgacgagcgcgacagcgtgcgtggcgaatacgccggccgtggcgccggtgtgcgcctgctggcaggcgagtgggaggacggcgccttcctgatggaggagtccgacgacggcacccgcgtatcgggcaactgggaaggcagcatcgacgccagcggcgccgtgcgcggcacctggaccgaatttaaatgcgcgc

SEQ ID NO: 27 - DNA, 2858 bp, synthetic construct
  source 1..2858: mol_type = other DNA
atccatttaaatggagttccagaccctgctcgactttatcgccgaagccgaactggaccgcgtcggctgcttcgcctactcgccggtggagggcgccaccgccaatgacctgccgggcgcgctgcccgacgaggtgcgcgaggaacgccgcgcccgcttcatggaagtggccgaagaggtctcggcgcgccgcctgcagcgcaaggtcggccagaccctgcgcgtgctggtggacgaggtcaaccaggatggcggcatcggccgttcgtccgcggatgcgccggaaatcgacggcctcgtctatatcgcgccgccggaacgccacgcccagcgctatcgcgccggcgagttcgtcgacgtgaagatcaccggcgccgatggccacgacctgtggggcgcggtctgaaacgggttgattaggtaaaagtacgctcgttcgatttcgtccgcgtcccgctatactgtgcggtgcaacataacctcatggagacaaagtccaattgcacgtgcagagagacaatcaaatcatgagccaaccatcttatggcccgctgttcgaggccctggcccactacaatgacaagctgctggccatggccaaggcccagacagagcgcaccgcccaggcgctgctgcagaccaatctggacgatctgggccaggtgctggagcagggcagccagcaaccctggcaactgatccaggcccagatgaactggtggcaggatcagctcaagctgatgcagcacaccctgctcaaaagcgcaggccagccgagcgagccggtgatcaccccggagcgcagcgatcgccgcttcaaggccgaggcctggagcgaacaacccatctatgactacctcaagcagtcctacctgctcaccgccaggcacctgctggcctcggtggatgccctggagggcgtcccccagaagagccgggagcggctgcgtttcttcacccgccagtacgtcagcgccatggcccccagcaacttcctggccaccaaccccgagctgctcaagctgaccctggagtccggcggccagaacctggtgcgcgggctggccctcttggccgaggatctggagcgcagcgccgatcagctcaacatccgcctgaccgacgaatccgccttcgagctcgggcgggatctggcgctcaccccgggccgggtggtgcagcgcaccgagctctatgagctgatccagtacagcccgactaccgagacggtgggcaagacacctgtgctgatagtgccccccttcatcaacaagtactacatcatggacatgcggccccagaactccctggtcgcctggctggtcgcccagggccagacggtgttcatgatctcctggcgcaacccgggcgtggcccaggcccaaatcgatctcgacgactacgtggtggacggggtcatcgccgccctggacggggtggaggcggccaccggcgagcgggaggtgcacggcatcggctactgcatcggcggcactgcactgtcgctcgccatgggctggctggcggcgcggcgccagaagcagcgagtgcgcaccgccaccctgttcactaccctgctggacttctcccagccaggggagctcggcatcttcatccacgagcccatcatagcggcgctcgaggcgcaaaatgaggccaagggcatcatggacgggcgccagctggctgtctccttcagcctgctgcgggagaacagcctctactggaactactacatcgacagctacctcaagggccagagcccggtggccttcgatctgctgcactggaacagcgacagcaccaatgtggcgggcaagacccacaacagcctgctgcgccgtctctacctggagaaccagctggtgaagggggagctcaagatccgcaacacccgcatcgatctcggcaaggtgaaaaccccggtactgctggtgtcggccgtggacgatcacatcgccctctggcagggcacctggcagggcatgaagctgtttggcggggagcagcgcttcctcctggcggagtccggccacatcgccggcatcatcaacccgccggccgccaacaagtacggcttctggcacaacggggccgaggccgagagcccggagagctggctggcaggggcgacgcaccagggcggctcctggtggcccgagatgatgggctttatccagaaccgtgacgaagggtcggagcccgtccccgcgcgggtgcccgaggaggggctggcccccgcccccggccactatgtcaaggtgcggctcaaccccgtgtttgcctgcccaacagaggaggacgccgcatgacctgccggcctggttcaaccagtcggcagccgactagtggttagccttgcgccttgcttcgctgacgaagaacctctgcgcgctcggcctggccgccgtgctcgcgctggcgggcacggcgcaggcagcgccggcgaccgagctgtcgaccggcccggttaacaccgggccagccggcggcgaaggcctgggcatcaaccaggccattcgcgacggcgaagcccggcgcggcggcacctcgctttccactggcgcgccaaaacccctggcgccgcggccggaatatgcgtcgctgccggtctacgtcggcaaggtcggcgaccagccggtgcggctgcgcctgggccccaagcctgacgagcgcgacagcgtgcgtggcgaatacgccggccgtggcgccggtgtgcgcctgctggcaggcgagtgggaggacggcgccttcctgatggaggagtccgacgacggcacccgcgtatcgggcaactgggaaggcagcatcgacgccagcggcgccgtgcgcggcacctggaccgaatttaaatccga

SEQ ID NO: 28 - DNA, 2800 bp, synthetic construct
  source 1..2800: mol_type = other DNA
atccatttaaatcccgggggtggatgcacagacccgcgagatctcggccaagctcgactccggcaagcacaccaccaccttcacgcggctctatcacctgccggccgaatggggcaccgtggacggccatcagggtgcgctgatcgattcgccgggcttccaggaattcggcctgtaccacctgagcgagggcatgctggagcgcgccttcccggagttccgcccgctgctgaccgggtgccgcttctacaactgccaccacgtcaacgagcccggctgcggcgtgctggccgcggtcgcctcgggagcgatctccgagcgccgccaccagctctacatgcagttgctgcacgaatccaaccagcagaagccgtggtaaggtaagcgcacctgggttacccggtgcgctgcccaattcgcgcaacgcaattaatgtgagttagctcactcattaggcaccccaggctttacactttatgcttccggctcgtatgttgtgtggaattgtgagcggataacaatttcacacaggaaacaattgcacgtgcagagagacaatcaaatcatgagccaaccatcttatggcccgctgttcgaggccctggcccactacaatgacaagctgctggccatggccaaggcccagacagagcgcaccgcccaggcgctgctgcagaccaatctggacgatctgggccaggtgctggagcagggcagccagcaaccctggcaactgatccaggcccagatgaactggtggcaggatcagctcaagctgatgcagcacaccctgctcaaaagcgcaggccagccgagcgagccggtgatcaccccggagcgcagcgatcgccgcttcaaggccgaggcctggagcgaacaacccatctatgactacctcaagcagtcctacctgctcaccgccaggcacctgctggcctcggtggatgccctggagggcgtcccccagaagagccgggagcggctgcgtttcttcacccgccagtacgtcagcgccatggcccccagcaacttcctggccaccaaccccgagctgctcaagctgaccctggagtccggcggccagaacctggtgcgcgggctggccctcttggccgaggatctggagcgcagcgccgatcagctcaacatccgcctgaccgacgaatccgccttcgagctcgggcgggatctggcgctcaccccgggccgggtggtgcagcgcaccgagctctatgagctgatccagtacagcccgactaccgagacggtgggcaagacacctgtgctgatagtgccccccttcatcaacaagtactacatcatggacatgcggccccagaactccctggtcgcctggctggtcgcccagggccagacggtgttcatgatctcctggcgcaacccgggcgtggcccaggcccaaatcgatctcgacgactacgtggtggacggggtcatcgccgccctggacggggtggaggcggccaccggcgagcgggaggtgcacggcatcggctactgcatcggcggcactgcactgtcgctcgccatgggctggctggcggcgcggcgccagaagcagcgagtgcgcaccgccaccctgttcactaccctgctggacttctcccagccaggggagctcggcatcttcatccacgagcccatcatagcggcgctcgaggcgcaaaatgaggccaagggcatcatggacgggcgccagctggctgtctccttcagcctgctgcgggagaacagcctctactggaactactacatcgacagctacctcaagggccagagcccggtggccttcgatctgctgcactggaacagcgacagcaccaatgtggcgggcaagacccacaacagcctgctgcgccgtctctacctggagaaccagctggtgaagggggagctcaagatccgcaacacccgcatcgatctcggcaaggtgaaaaccccggtactgctggtgtcggccgtggacgatcacatcgccctctggcagggcacctggcagggcatgaagctgtttggcggggagcagcgcttcctcctggcggagtccggccacatcgccggcatcatcaacccgccggccgccaacaagtacggcttctggcacaacggggccgaggccgagagcccggagagctggctggcaggggcgacgcaccagggcggctcctggtggcccgagatgatgggctttatccagaaccgtgacgaagggtcggagcccgtccccgcgcgggtgcccgaggaggggctggcccccgcccccggccactatgtcaaggtgcggctcaaccccgtgtttgcctgcccaacagaggaggacgccgcatgacctgccggcctggttcaaccagtcggcagccgactagtatgaaactgctgctgtccgccacttccctcgtccatgcagcccattgccggaacgtcctgcgggcggccggcatccgggcggaattgcgcaatacctggctggccggcgcgaccggcgagatcccgttccgggagagtgcgccacaggtgtggctggtcgatgacgagatggaagcgcaggcgtgggcggtgctcaatgccgccgccaacccggcgccggggccgagctggcaatgccgccactgcctggaatggcacgaggcccagttcggggcctgctggcgctgcggcgcggcccgcgactagcgcgccgccccctttttgacgctggtcagccgacccagagcgccagcgacagcatcgccagcagcagcatccacagcaccaccgcgcgccatacatttaaatccga

SEQ ID NO: 29 - DNA, 2840 bp, synthetic construct
  source 1..2840: mol_type = other DNA
atccatttaaatcgatcgcccggcgcctggaagagctcggggccgatacgcgcgccatcgtggtggtggaagtgggcaatgccgcgtcgcagattcctctgccgacgcaggcgcaatgcgatgtgcactggctgcatcgtgacgatgcgctggaaggcagcctgctggaaggggtgctacgcaagctcacgctgccgcgcggcgagggttatgtgtgggccgctggtgaagccgcggcgatgaaagcggtgcgccagtacctggtcagcgaacgcggtgtcgacaagcgccgtatccgcgcgtcggcgtactggaagcgtggcgcttcggcggtgcatgagacgctggacgactgaagcgggcggggtgccggtaagatagtgcgaccgccatccgccagggagaccctgcccaattctgcttctggcgtcaggcagccatcggaagctgtggtatggctgtgcaggtcgtaaatcactgcataattcgtgtcgctcaaggcgcactcccgttctggataatgttttttgcgccgacatcataacggttctggcaaatattctgaaatgagctgttgacaattaatcatcgaactagttaactagtacgcaagttcacagcggataacaatttcacacaggaaacaattgcacgtgcagagagacaatcaaatcatgcagcagtttgtcaattccctgtcgctcggccaggaccagtccgatgccccccatccgctgaccggcgcctggtcgcagctgatgagccagaccaatcagctcttgcagctgcaatccagcctctaccaacagcaattgggcttgtggacgcaattcctcggccaaaccgccggcaacgacgcttccgcgccgtcggccaagccgagcgaccgccgcttcgcctcgccggagtgggatgagcatccgttctacagcttcctcaagcagagctatctgcaaacctccaagtggatgatggagctggtggacaagacccagatcgacgaaagcgctaaggacaagctgtccttcgccactcgccagtacctggatgccatggcgcccagcaacttcatgctgaccaaccccgacgtggtcaaacgcgccatcgaaacccagggcgaaagcctggtggaaggcatgaagaacatgatggaggacatccagaagggccatatctcgatgtccgacgagagcaagttccaaatcggcaaaaacctggtggtgacgccgggcgaggtggtgttccgcaatgaactgatcgagctgatccagtacacgccgaccaccgaaaaagtccacgaaaagcccttgctgtttgtcccgccgtgcatcaacaagtactacctgatggatctgcagccggacaactccatggtgcgccacttcgtcggccagggttaccgcgttttcctggtcagctggcgttccgccgtgcccgagatgaagaacttcacttgggagacctacatcgagaaaggcgtgttcgccgcggccgaagcggttcagaagatcaccaagcagccgaccatgaacgcgctgggcttctgcgtgggcggcgtgatcctcactaccgcgctgtgcgtggcccaggccaagggtctgaaatacttcgactccgccaccttcatgacgtcgctgatcgaccacgccgaaccgggcgagatctccttcttcatcgacgaggcgctggtagccagccgcgaagccaaaatggcggccggcggcatcatcagcggcaaggaaatcggacgcactttcgccagcctgcgcgccaacgacctggtgtggaactacgtcgtcaacaactacctgctgggcaagaccccggcgccgttcgacctgctgtactggaacaacgacgcggtggacctgccgctgccgatgcacaccttcatgctgcggcagttctacatcaacaacgcgctgatcaccccgggcgccattacgctgtgcggcgtcccgatcgacatctccaagatcgacatcccggtgtatatgttcgccgcgcgcgaagaccacatcgtgctgtggagttccgcctactccggcctgaaatatctgagcggcacgccaagccgccgctttgtcctgggcgcatccggccacatctggggctcgatcaaccccgtcaccaaggataagcgcaactactggaccaacgagcagctgccggtgaatccggaagaatggctggagggcgcgcaaagccatccaggcagctggtggaaggactgggacgcctggctggccccgcaatccggaaaacaggttccggcgcccaagatgctgggcagcaaggagttccccccgctgcagcctgcgccgggcagctatgtgctcgccaaggcgatgcctcccgtcgccgccgccttgaactgacctgccggcctggttcaaccagtcggcagccggaattgatcgatactagtgtgcagccttcgcccacctttcgccgcttcacgatcagccggcgcttcgcgctggcctgcgcctgcgcagcgttgctggcggcctgtgcgccggactccgtgcgcaatatccaggccaagggcttcaatgcctatctcgattcgctgcagaccgcttgccccaacatggtggttggctccagcaatatcagcgactggctgcgcaccagtggcagcaggggcgacgacaactacgtctactggctggaccagacctcgcggctctactaccagcgcatctcgccaacgcagtatcgggattcggtcagcgcggcgcttggcggcaagtcagattcgcgcgcgctggactgcatcgtgcgcaacctgccgccggaccggccgacgcgtccgccgggcggcaatttaaatccga

SEQ ID NO: 30 - DNA, 2677 bp, synthetic construct
  source 1..2677: mol_type = other DNA
atccatttaaatcgatcgcccggcgcctggaagagctcggggccgatacgcgcgccatcgtggtggtggaagtgggcaatgccgcgtcgcagattcctctgccgacgcaggcgcaatgcgatgtgcactggctgcatcgtgacgatgcgctggaaggcagcctgctggaaggggtgctacgcaagctcacgctgccgcgcggcgagggttatgtgtgggccgctggtgaagccgcggcgatgaaagcggtgcgccagtacctggtcagcgaacgcggtgtcgacaagcgccgtatccgcgcgtcggcgtactggaagcgtggcgcttcggcggtgcatgagacgctggacgactgaagcgggcggggtgccggtaagatagtgcgaccgccatccgccagggagaccctgcccaattgcacgtgcagagagacaatcaaatcatgagccaaccatcttatggcccgctgttcgaggccctggcccactacaatgacaagctgctggccatggccaaggcccagacagagcgcaccgcccaggcgctgctgcagaccaatctggacgatctgggccaggtgctggagcagggcagccagcaaccctggcaactgatccaggcccagatgaactggtggcaggatcagctcaagctgatgcagcacaccctgctcaaaagcgcaggccagccgagcgagccggtgatcaccccggagcgcagcgatcgccgcttcaaggccgaggcctggagcgaacaacccatctatgactacctcaagcagtcctacctgctcaccgccaggcacctgctggcctcggtggatgccctggagggcgtcccccagaagagccgggagcggctgcgtttcttcacccgccagtacgtcagcgccatggcccccagcaacttcctggccaccaaccccgagctgctcaagctgaccctggagtccggcggccagaacctggtgcgcgggctggccctcttggccgaggatctggagcgcagcgccgatcagctcaacatccgcctgaccgacgaatccgccttcgagctcgggcgggatctggcgctcaccccgggccgggtggtgcagcgcaccgagctctatgagctgatccagtacagcccgactaccgagacggtgggcaagacacctgtgctgatagtgccccccttcatcaacaagtactacatcatggacatgcggccccagaactccctggtcgcctggctggtcgcccagggccagacggtgttcatgatctcctggcgcaacccgggcgtggcccaggcccaaatcgatctcgacgactacgtggtggacggggtcatcgccgccctggacggggtggaggcggccaccggcgagcgggaggtgcacggcatcggctactgcatcggcggcactgcactgtcgctcgccatgggctggctggcggcgcggcgccagaagcagcgagtgcgcaccgccaccctgttcactaccctgctggacttctcccagccaggggagctcggcatcttcatccacgagcccatcatagcggcgctcgaggcgcaaaatgaggccaagggcatcatggacgggcgccagctggctgtctccttcagcctgctgcgggagaacagcctctactggaactactacatcgacagctacctcaagggccagagcccggtggccttcgatctgctgcactggaacagcgacagcaccaatgtggcgggcaagacccacaacagcctgctgcgccgtctctacctggagaaccagctggtgaagggggagctcaagatccgcaacacccgcatcgatctcggcaaggtgaaaaccccggtactgctggtgtcggccgtggacgatcacatcgccctctggcagggcacctggcagggcatgaagctgtttggcggggagcagcgcttcctcctggcggagtccggccacatcgccggcatcatcaacccgccggccgccaacaagtacggcttctggcacaacggggccgaggccgagagcccggagagctggctggcaggggcgacgcaccagggcggctcctggtggcccgagatgatgggctttatccagaaccgtgacgaagggtcggagcccgtccccgcgcgggtgcccgaggaggggctggcccccgcccccggccactatgtcaaggtgcggctcaaccccgtgtttgcctgcccaacagaggaggacgccgcatgacctgccggcctggttcaaccagtcggcagccgactagtgtgcagccttcgcccacctttcgccgcttcacgatcagccggcgcttcgcgctggcctgcgcctgcgcagcgttgctggcggcctgtgcgccggactccgtgcgcaatatccaggccaagggcttcaatgcctatctcgattcgctgcagaccgcttgccccaacatggtggttggctccagcaatatcagcgactggctgcgcaccagtggcagcaggggcgacgacaactacgtctactggctggaccagacctcgcggctctactaccagcgcatctcgccaacgcagtatcgggattcggtcagcgcggcgcttggcggcaagtcagattcgcgcgcgctggactgcatcgtgcgcaacctgccgccggaccggccgacgcgtccgccgggcggcaatttaaatccga

SEQ ID NO: 31 - DNA, 139 bp, synthetic construct
  source 1..139: mol_type = other DNA
gcgcgaattcgcgcaacgcaattaatgtgagttagctcactcattaggcaccccaggctttacactttatgcttccggctcgtataatgtgtggaattgtgagcggataacaatttcacacaggaaacaattgcacgtg

SEQ ID NO: 32 - DNA, 1780 bp, synthetic construct
  source 1..1780: mol_type = other DNA
gaaagaattccacgtgcagagagacaatcaaatcatgcagcagtttgtcaattccctgtcgctcggccaggaccagtccgatgccccccatccgctgaccggcgcctggtcgcagctgatgagccagaccaatcagctcttgcagctgcaatccagcctctaccaacagcaattgggcttgtggacgcaattcctcggccaaaccgccggcaacgacgcttccgcgccgtcggccaagccgagcgaccgccgcttcgcctcgccggagtgggatgagcatccgttctacagcttcctcaagcagagctatctgcaaacctccaagtggatgatggagctggtggacaagacccagatcgacgaaagcgctaaggacaagctgtccttcgccactcgccagtacctggatgccatggcgcccagcaacttcatgctgaccaaccccgacgtggtcaaacgcgccatcgaaacccagggcgaaagcctggtggaaggcatgaagaacatgatggaggacatccagaagggccatatctcgatgtccgacgagagcaagttccaaatcggcaaaaacctggtggtgacgccgggcgaggtggtgttccgcaatgaactgatcgagctgatccagtacacgccgaccaccgaaaaagtccacgaaaagcccttgctgtttgtcccgccgtgcatcaacaagtactacctgatggatctgcagccggacaactccatggtgcgccacttcgtcggccagggttaccgcgttttcctggtcagctggcgttccgccgtgcccgagatgaagaacttcacttgggagacctacatcgagaaaggcgtgttcgccgcggccgaagcggttcagaagatcaccaagcagccgaccatgaacgcgctgggcttctgcgtgggcggcgtgatcctcactaccgcgctgtgcgtggcccaggccaagggtctgaaatacttcgactccgccaccttcatgacgtcgctgatcgaccacgccgaaccgggcgagatctccttcttcatcgacgaggcgctggtagccagccgcgaagccaaaatggcggccggcggcatcatcagcggcaaggaaatcggacgcactttcgccagcctgcgcgccaacgacctggtgtggaactacgtcgtcaacaactacctgctgggcaagaccccggcgccgttcgacctgctgtactggaacaacgacgcggtggacctgccgctgccgatgcacaccttcatgctgcggcagttctacatcaacaacgcgctgatcaccccgggcgccattacgctgtgcggcgtcccgatcgacatctccaagatcgacatcccggtgtatatgttcgccgcgcgcgaagaccacatcgtgctgtggagttccgcctactccggcctgaaatatctgagcggcacgccaagccgccgctttgtcctgggcgcatccggccacatctggggctcgatcaaccccgtcaccaaggataagcgcaactactggaccaacgagcagctgccggtgaatccggaagaatggctggagggcgcgcaaagccatccaggcagctggtggaaggactgggacgcctggctggccccgcaatccggaaaacaggttccggcgcccaagatgctgggcagcaaggagttccccccgctgcagcctgcgccgggcagctatgtgctcgccaaggcgatgcctcccgtcgccgccgccttgaactgacctgccggcctggttcaaccagtcggcagccgactagtggat

SEQ ID NO: 33 - DNA, 2982 bp, synthetic construct
  source 1..2982: mol_type = other DNA
atccatttaaatggagttccagaccctgctcgactttatcgccgaagccgaactggaccgcgtcggctgcttcgcctactcgccggtggagggcgccaccgccaatgacctgccgggcgcgctgcccgacgaggtgcgcgaggaacgccgcgcccgcttcatggaagtggccgaagaggtctcggcgcgccgcctgcagcgcaaggtcggccagaccctgcgcgtgctggtggacgaggtcaaccaggatggcggcatcggccgttcgtccgcggatgcgccggaaatcgacggcctcgtctatatcgcgccgccggaacgccacgcccagcgctatcgcgccggcgagttcgtcgacgtgaagatcaccggcgccgatggccacgacctgtggggcgcggtctgaaacgggttgattaggtaaaagtacgctcgttcgatttcgtccgcgtcccgctatactgtgcggtgcaacataacctcatggagacaaagtccaattggcgcaacgcaattaatgtgagttagctcactcattaggcaccccaggctttacacctttatgcttccggctcgtatgttgtgtggaattgtgagcggataacaatttcacacaggaaacaattgcacgtgcagagagacaatcaaatcatgagccaaccatcttatggcccgctgttcgaggccctggcccactacaatgacaagctgctggccatggccaaggcccagacagagcgcaccgcccaggcgctgctgcagaccaatctggacgatctgggccaggtgctggagcagggcagccagcaaccctggcaactgatccaggcccagatgaactggtggcaggatcagctcaagctgatgcagcacaccctgctcaaaagcgcaggccagccgagcgagccggtgatcaccccggagcgcagcgatcgccgcttcaaggccgaggcctggagcgaacaacccatctatgactacctcaagcagtcctacctgctcaccgccaggcacctgctggcctcggtggatgccctggagggcgtcccccagaagagccgggagcggctgcgtttcttcacccgccagtacgtcagcgccatggcccccagcaacttcctggccaccaaccccgagctgctcaagctgaccctggagtccggcggccagaacctggtgcgcgggctggccctcttggccgaggatctggagcgcagcgccgatcagctcaacatccgcctgaccgacgaatccgccttcgagctcgggcgggatctggcgctcaccccgggccgggtggtgcagcgcaccgagctctatgagctgatccagtacagcccgactaccgagacggtgggcaagacacctgtgctgatagtgccccccttcatcaacaagtactacatcatggacatgcggccccagaactccctggtcgcctggctggtcgcccagggccagacggtgttcatgatctcctggcgcaacccgggcgtggcccaggcccaaatcgatctcgacgactacgtggtggacggggtcatcgccgccctggacggggtggaggcggccaccggcgagcgggaggtgcacggcatcggctactgcatcggcggcactgcactgtcgctcgccatgggctggctggcggcgcggcgccagaagcagcgagtgcgcaccgccaccctgttcactaccctgctggacttctcccagccaggggagctcggcatcttcatccacgagcccatcatagcggcgctcgaggcgcaaaatgaggccaagggcatcatggacgggcgccagctggctgtctccttcagcctgctgcgggagaacagcctctactggaactactacatcgacagctacctcaagggccagagcccggtggccttcgatctgctgcactggaacagcgacagcaccaatgtggcgggcaagacccacaacagcctgctgcgccgtctctacctggagaaccagctggtgaagggggagctcaagatccgcaacacccgcatcgatctcggcaaggtgaaaaccccggtactgctggtgtcggccgtggacgatcacatcgccctctggcagggcacctggcagggcatgaagctgtttggcggggagcagcgcttcctcctggcggagtccggccacatcgccggcatcatcaacccgccggccgccaacaagtacggcttctggcacaacggggccgaggccgagagcccggagagctggctggcaggggcgacgcaccagggcggctcctggtggcccgagatgatgggctttatccagaaccgtgacgaagggtcggagcccgtccccgcgcgggtgcccgaggaggggctggcccccgcccccggccactatgtcaaggtgcggctcaaccccgtgtttgcctgcccaacagaggaggacgccgcatgacctgccggcctggttcaaccagtcggcagccgactagtggttagccttgcgccttgcttcgctgacgaagaacctctgcgcgctcggcctggccgccgtgctcgcgctggcgggcacggcgcaggcagcgccggcgaccgagctgtcgaccggcccggttaacaccgggccagccggcggcgaaggcctgggcatcaaccaggccattcgcgacggcgaagcccggcgcggcggcacctcgctttccactggcgcgccaaaacccctggcgccgcggccggaatatgcgtcgctgccggtctacgtcggcaaggtcggcgaccagccggtgcggctgcgcctgggccccaagcctgacgagcgcgacagcgtgcgtggcgaatacgccggccgtggcgccggtgtgcgcctgctggcaggcgagtgggaggacggcgccttcctgatggaggagtccgacgacggcacccgcgtatcgggcaactgggaaggcagcatcgacgccagcggcgccgtgcgcggcacctggaccgaatttaaatccga

SEQ ID NO: 34 - DNA, 2793 bp, synthetic construct
  source 1..2793: mol_type = other DNA
atccatttaaatcaggcacttgaagcacgcgacggcaagcggcttgcggccatcctgcgccagcacctcctggacaagcgcgacgcggtgctgctgatccaggcaggcgatgccgttggcacgccccaggcataggacgctggcgccaccctcaccccaagaatccgaatagccccatcagcattctttgccccgctgtcaccacggtgacaaccccggttcttactctgcgagcgcattgcggcaaacgcaatccgccatgcggcacctgccgcagcgcacaacaacgcagatgaacaggggaatcaaagatggcagggaaccttgcaccggacaggctggcggggatgtcgcgcggccgtcaattgtgcttctggcgtcaggcagccatcggaagctgtggtatggctgtgcaggtcgtaaatcactgcataattcgtgtcgctcaaggcgcactcccgttctggataatgttttttgcgccgacatcataacggttctggcaaatattctgaaatgagctgttgacaattaatcatcgaactagttaactagtacgcaagttcacagcggataacaatttcacacaggaaacaattcacgtgcagagagacaatcaaatcatgagccaaccatcttatggcccgctgttcgaggccctggcccactacaatgacaagctgctggccatggccaaggcccagacagagcgcaccgcccaggcgctgctgcagaccaatctggacgatctgggccaggtgctggagcagggcagccagcaaccctggcagctgatccaggcccagatgaactggtggcaggatcagctcaagctgatgcagcacaccctgctcaaaagcgcaggccagccgagcgagccggtgatcaccccggagcgcagcgatcgccgcttcaaggccgaggcctggagcgaacaacccatctatgactacctcaagcagtcctacctgctcaccgccaggcacctgctggcctcggtggatgccctggagggcgtcccccagaagagccgggagcggctgcgtttcttcacccgccagtacgtcagcgccatggcccccgccaacttccttgccaccaatcccgaggcgcagcgcctgctgatcgagtcgggcggcgaatcgctgcgtgccggcgtgcgcaacatgatggaagacctgacacgcggcaagatctcgcagaccgacgagagcgcgtttgaggtcggccgcaatgtcgcggtgaccgaaggcgccgtggtcttcgagaacgagtacttccagctgttgcagtacaagccgctgaccgacaaggtgcacgcgcgcccgctgctgatggtgccgccgtgcatcaacaagtactacatcctggacctgcagccggagagctcgctggtgcgccatgtggtggagcagggacatacggtgtttctggtgtcgtggcgcaatccggacgccagcatggccggcagcacctgggacgactacatcgagcacgcggccatccgcgccatcgaagtcgcgcgcgacatcagcggccaggacaagatcaacgtgctcggcttctgcgtgggcggcaccattgtctcgaccgcgctggcggtgctggccgcgcgcggcgagcacccggccgccagcgtcacgctgctgaccacgctgctggactttgccgacacgggcatcctcgacgtctttgtcgacgagggccatgtgcagttgcgcgaggccacgctgggcggcggcgccggcgcgccgtgcgcgctgctgcgcggccttgagctggccaataccttctcgttcttgcgcccgaacgacctggtgtggaactacgtggtcgacaactacctgaagggcaacacgccggtgccgttcgacctgctgttctggaacggcgacgccaccaacctgccggggccgtggtactgctggtacctgcgccacacctacctgcagaacgagctcaaggtaccgggcaagctgaccgtgtgcggcgtgccggtggacctggccagcatcgacgtgccgacctatatctacggctcgcgcgaagaccatatcgtgccgtggaccgcggcctatgcctcgaccgcgctgctggcgaacaagctgcgcttcgtgctgggtgcgtcgggccatatcgccggtgtgatcaacccgccggccaagaacaagcgcagccactggactaacgatgcgctgccggagtcgccgcagcaatggctggccggcgccatcgagcatcacggcagctggtggccggactggaccgcatggctggccgggcaggccggcgcgaaacgcgccgcgcccgccaactatggcaatgcgcgctatcgcgcaatcgaacccgcgcctgggcgatacgtcaaagccaaggcatgacctgccggcctggttcaaccagtcggcagccggaattgatcgatactagtatccggccggagcccgtttcgtcacggaacgggttcctcaccgacccttcccccccgcccgatcccctgcaggagattgacaccatgactttccgaccttccaccctggcgcggccgcactggctcgccgccgtgctgatgtgcgcagcgctcgccgcctgcggcggcgactccggcgacagccccaccggctcgcccaacgcggcaccgatcacgccgggtgccccgggtaccggcggcaaccccggccaggggaatggcagcgaccagcctggcgagacgcccgccgtgaagccgcagctgcgctgcgcaccctgaagccgggcctggcccgtctcccctccagaaacatttaaatccga

SEQ ID NO: 35 - DNA, 2793 bp, synthetic construct; identical to SEQ ID NO: 34
  source 1..2793: mol_type = other DNA

SEQ ID NO: 36 - DNA, 1834 bp, synthetic construct
  source 1..1834: mol_type = other DNA
gaaacaattgcacgtgcagagagacaatcaaatcatgagccaaccatcttatggcccgctgttcgaggccctggcccactacaatgacaagctgctggccatggccaaggcccagacagagcgcaccgcccaggcgctgctgcagaccaatctggacgatctgggccaggtgctggagcagggcagccagcaaccctggcaactgatccaggcccagatgaactggtggcaggatcagctcaagctgatgcagcacaccctgctcaaaagcgcaggccagccgagcgagccggtgatcaccccggagcgcagcgatcgccgcttcaaggccgaggcctggagcgaacaacccatctatgactacctcaagcagtcctacctgctcaccgccaggcacctgctggcctcggtggatgccctggagggcgtcccccagaagagccgggagcggctgcgtttcttcacccgccagtacgtcagcgccatggcccccgccaacttccttgccaccaatcccgaggcgcagcgcctgctgatcgagtcgggcggcgaatcgctgcgtgccggcgtgcgcaacatgatggaagacctgacacgcggcaagatctcgcagaccgacgagagcgcgtttgaggtcggccgcaatgtcgcggtgaccgaaggcgccgtggtcttcgagaacgagtacttccagctgttgcagtacaagccgctgaccgacaaggtgcacgcgcgcccgctgctgatggtgccgccgtgcatcaacaagtactacatcctggacctgcagccggagagctcgctggtgcgccatgtggtggagcagggacatacggtgtttctggtgtcgtggcgcaatccggacgccagcatggccggcagcacctgggacgactacatcgagcacgcggccatccgcgccatcgaagtcgcgcgcgacatcagcggccaggacaagatcaacgtgctcggcttctgcgtgggcggcaccattgtctcgaccgcgctggcggtgctggccgcgcgcggcgagcacccggccgccagcgtcacgctgctgaccacgctgctggactttgccgacacgggcatcctcgacgtctttgtcgacgagggccatgtgcagttgcgcgaggccacgctgggcggcggcgccggcgcgccgtgcgcgctgctgcgcggccttgagctggccaataccttctcgttcttgcgcccgaacgacctggtgtggaactacgtggtcgacaactacctgaagggcaacacgccggtgccgttcgacctgctgttctggaacggcgacgccaccaacctgccggggccgtggtactgctggtacctgcgccacacctacctgcagaacgagctcaaggtaccgggcaagctgaccgtgtgcggcgtgccggtggacctggccagcatcgacgtgccgacctatatctacggctcgcgcgaagaccatatcgtgccgtggaccgcggcctatgcctcgaccgcgctgctggcgaacaagctgcgcttcgtgctgggtgcgtcgggccatatcgccggtgtgatcaacccgccggccaagaacaagcgcagccactggactaacgatgcgctgccggagtcgccgcagcaatggctggccggcgccatcgagcatcacggcagctggtggccggactggaccgcatggctggccgggcaggccggcgcgaaacgcgccgcgcccgccaactatggcaatgcgcgctatcgcgcaatcgaacccgcgcctgggcgatacgtcaaagccaaggcatgacctgccggcctggttcaaccagtcggcagccgactagtggat

SEQ ID NO: 37 - DNA, 246 bp, synthetic construct
  source 1..246: mol_type = other DNA
gcgccaattgtgcttctggcgtcaggcagccatcggaagctgtggtatggctgtgcaggtcgtaaatcactgcataattcgtgtcgctcaaggcgcactcccgttctggataatgttttttgcgccgacatcataacggttctggcaaatattctgaaatgagctgttgacaattaatcatcgaactagttaactagtacgcaagttcacagcggataacaatttcacacaggaaacaattgcacg

SEQ ID NO: 38 - DNA, 1846 bp, synthetic construct
  source 1..1846: mol_type = other DNA
gcgccaattgcacgtgcagagagacaatcaaatcatgagccaaccatcttatggcccgctgttcgaggccctggcccactacaatgacaagctgctggccatggccaaggcccagacagagcgcaccgcccaggcgctgctgcagaccaatctggacgatctgggccaggtgctggagcagggcagccagcaaccctggcaactgatccaggcccagatgaactggtggcaggatcagctcaagctgatgcagcacaccctgctcaaaagcgcaggccagccgagcgagccggtgatcaccccggagcgcagcgatcgccgcttcaaggccgaggcctggagcgaacaacccatctatgactacctcaagcagtcctacctgctcaccgccaggcacctgctggcctcggtggatgccctggagggcgtcccccagaagagccgggagcggctgcgtttcttcacccgccagtacgtcagcgccatggcccccgccaacttccttgccaccaatcccgaggcgcagcgcctgctgatcgagtcgggcggcgaatcgctgcgtgccggcgtgcgcaacatgatggaagacctgacacgcggcaagatctcgcagaccgacgagagcgcgtttgaggtcggccgcaatgtcgcggtgaccgaaggcgccgtggtcttcgagaacgagtacttccagctgttgcagtacaagccgctgaccgacaaggtgcacgcgcgcccgctgctgatggtgccgccgtgcatcaacaagtactacatcctggacctgcagccggagagctcgctggtgcgccatgtggtggagcagggacatacggtgtttctggtgtcgtggcgcaatccggacgccagcatggccggcagcacctgggacgactacatcgagcacgcggccatccgcgccatcgaagtcgcgcgcgacatcagcggccaggacaagatcaacgtgctcggcttctgcgtgggcggcaccattgtctcgaccgcgctggcggtgctggccgcgcgcggcgagcacccggccgccagcgtcacgctgctgaccacgctgctggactttgccgacacgggcatcctcgacgtctttgtcgacgagggccatgtgcagttgcgcgaggccacgctgggcggcggcgccggcgcgccgtgcgcgctgctgcgcggccttgagctggccaataccttctcgttcttgcgcccgaacgacctggtgtggaactacgtggtcgacaactacctgaagggcaacacgccggtgccgttcgacctgctgttctggaacggcgacgccaccaacctgccggggccgtggtactgctggtacctgcgccacacctacctgcagaacgagctcaaggtaccgggcaagctgaccgtgtgcggcgtgccggtggacctggccagcatcgacgtgccgacctatatctacggctcgcgcgaagaccatatcgtgccgtggaccgcggcctatgcctcgaccgcgctgctggcgaacaagctgcgcttcgtgctgggtgcgtcgggccatatcgccggtgtgatcaacccgccggccaagaacaagcgcagccactggactaacgatgcgctgccggagtcgccgcagcaatggctggccggcgccatcgagcatcacggcagctggtggccggactggaccgcatggctggccgggcaggccggcgcgaaacgcgccgcgcccgccaactatggcaatgcgcgctatcgcgcaatcgaacccgcgcctgggcgatacgtcaaagccaaggcatgacctgccggcctggttcaaccagtcggcagccggaattgatcgatactagtgcgc

SEQ ID NO: 39 - DNA, 2982 bp, synthetic construct
  source 1..2982: mol_type = other DNA
atccatttaaatggagttccagaccctgctcgactttatcgccgaagccgaactggaccgcgtcggctgcttcgcctactcgccggtggagggcgccaccgccaatgacctgccgggcgcgctgcccgacgaggtgcgcgaggaacgccgcgcccgcttcatggaagtggccgaagaggtctcggcgcgccgcctgcagcgcaaggtcggccagaccctgcgcgtgctggtggacgaggtcaaccaggatggcggcatcggccgttcgtccgcggatgcgccggaaatcgacggcctcgtctatatcgcgccgccggaacgccacgcccagcgctatcgcgccggcgagttcgtcgacgtgaagatcaccggcgccgatggccacgacctgtggggcgcggtctgaaacgggttgattaggtaaaagtacgctcgttcgatttcgtccgcgtcccgctatactgtgcggtgcaacataacctcatggagacaaagtccaattggcgcaacgcaattaatgtgagttagctcactcattaggcaccccaggctttacacctttatgcttccggctcgtatgttgtgtggaattgtgagcggataacaatttcacacaggaaacaattgcacgtgcagagagacaatcaaatcatgagccaaccatcttatggcccgctgttcgaggccctggcccactacaatgacaagctgctggccatggccaaggcccagacagagcgcaccgcccaggcgctgctgcagaccaatctggacgatctgggccaggtgctggagcagggcagccagcaaccctggcaactgatccaggcccagatgaactggtggcaggatcagctcaagctgatgcagcacaccctgctcaaaagcgcaggccagccgagcgagccggtgatcaccccggagcgcagcgatcgccgcttcaaggccgaggcctggagcgaacaacccatctatgactacctcaagcagtcctacctgctcaccgccaggcacctgctggcctcggtggatgccctggagggcgtcccccagaagagccgggagcggctgcgtttcttcacccgccagtacgtcagcgccatggcccccagcaacttcctggccaccaaccccgagctgctcaagctgaccctggagtccggcggccagaacctggtgcgcgggctggccctcttggccgaggatctggagcgcagcgccgatcagctcaacatccgcctgaccgacgaatccgccttcgagctcgggcgggatctggcgctcaccccgggccgggtggtgcagcgcaccgagctctatgagctgatccagtacagcccgactaccgagacggtgggcaagacacctgtgctgatagtgccccccttcatcaacaagtactacatcatggacatgcggccccagaactccctggtcgcctggctggtcgcccagggccagacggtgttcatgatctcctggcgcaacccgggcgtggcccaggcccaaatcgatctcgacgactacgtggtggacggggtcatcgccgccctggacggggtggaggcggccaccggcgagcgggaggtgcacggcatcggctactgcatcggcggcactgcactgtcgctcgccatgggctggctggcggcgcggcgccagaagcagcgagtgcgcaccgccaccctgttcactaccctgctggacttctcccagccaggggagctcggcatcttcatccacgagcccatcatagcggcgctcgaggcgcaaaatgaggccaagggcatcatggacgggcgccagctggctgtcggcttcagcctgctgcgggagaacagcctctactggaactactacatcgacagctacctcaagggccagagcccggtggccttcgatctgctgcactggaacagcgacagcaccaatgtggcgggcaagacccacaacagcctgctgcgccgtctctacctggagaaccagctggtgaagggggagctcaagatccgcaacacccgcatcgatctcggcaaggtgaaaaccccggtactgctggtgtcggccgtggacgatcacatcgccctctggcagggcacctggcagggcatgaagctgtttggcggggagcagcgcttcctcctggcggagtccggccacatcgccggcatcatcaacccgccggccgccaacaagtacggcttctggcacaacggggccgaggccgagagcccggagagctggctggcaggggcgacgcaccagggcggctcctggtggcccgagatgatgggctttatccagaaccgtgacgaagggtcggagcccgtccccgcgcgggtgcccgaggaggggctggcccccgcccccggccactatgtcaaggtgcggctcaaccccgtgtttgcctgcccaacagaggaggacgccgcatgacctgccggcctggttcaaccagtcggcagccgactagtggttagccttgcgccttgcttcgctgacgaagaacctctgcgcgctcggcctggccgccgtgctcgcgctggcgggcacggcgcaggcagcgccggcgaccgagctgtcgaccggcccggttaacaccgggccagccggcggcgaaggcctgggcatcaaccaggccattcgcgacggcgaagcccggcgcggcggcacctcgctttccactggcgcgccaaaacccctggcgccgcggccggaatatgcgtcgctgccggtctacgtcggcaaggtcggcgaccagccggtgcggctgcgcctgggccccaagcctgacgagcgcgacagcgtgcgtggcgaatacgccggccgtggcgccggtgtgcgcctgctggcaggcgagtgggaggacggcgccttcctgatggaggagtccgacgacggcacccgcgtatcgggcaactgggaaggcagcatcgacgccagcggcgccgtgcgcggcacctggaccgaatttaaatccga

SEQ ID NO: 40 - DNA, 2858 bp, synthetic construct
  source 1..2858: mol_type = other DNA
atccatttaaatggagttccagaccctgctcgactttatcgccgaagccgaactggaccgcgtcggctgcttcgcctactcgccggtggagggcgccaccgccaatgacctgccgggcgcgctgcccgacgaggtgcgcgaggaacgccgcgcccgcttcatggaagtggccgaagaggtctcggcgcgccgcctgcagcgcaaggtcggccagaccctgcgcgtgctggtggacgaggtcaaccaggatggcggcatcggccgttcgtccgcggatgcgccggaaatcgacggcctcgtctatatcgcgccgccggaacgccacgcccagcgctatcgcgccggcgagttcgtcgacgtgaagatcaccggcgccgatggccacgacctgtggggcgcggtctgaaacgggttgattaggtaaaagtacgctcgttcgatttcgtccgcgtcccgctatactgtgcggtgcaacataacctcatggagacaaagtccaattgcacgtgcagagagacaatcaaatcatgagccaaccatcttatggcccgctgttcgaggccctggcccactacaatgacaagctgctggccatggccaaggcccagacagagcgcaccgcccaggcgctgctgcagaccaatctggacgatctgggccaggtgctggagcagggcagccagcaaccctggcaactgatccaggcccagatgaactggtggcaggatcagctcaagctgatgcagcacaccctgctcaaaagcgcaggccagccgagcgagccggtgatcaccccggagcgcagcgatcgccgcttcaaggccgaggcctggagcgaacaacccatctatgactacctcaagcagtcctacctgctcaccgccaggcacctgctggcctcggtggatgccctggagggcgtcccccagaagagccgggagcggctgcgtttcttcacccgccagtacgtcagcgccatggcccccagcaacttcctggccaccaaccccgagctgctcaagctgaccctggagtccggcggccagaacctggtgcgcgggctggccctcttggccgaggatctggagcgcagcgccgatcagctcaacatccgcctgaccgacgaatccgccttcgagctcgggcgggatctggcgctcaccccgggccgggtggtgcagcgcaccgagctctatgagctgatccagtacagcccgactaccgagacggtgggcaagacacctgtgctgatagtgccccccttcatcaacaagtactacatcatggacatgcggccccagaactccctggtcgcctggctggtcgcccagggccagacggtgttcatgatctcctggcgcaacccgggcgtggcccaggcccaaatcgatctcgacgactacgtggtggacggggtcatcgccgccctggacggggtggaggcggccaccggcgagcgggaggtgcacggcatcggctactgcatcggcggcactgcactgtcgctcgccatgggctggctggcggcgcggcgccagaagcagcgagtgcgcaccgccaccctgttcactaccctgctggacttctcccagccaggggagctcggcatcttcatccacgagcccatcatagcggcgctcgaggcgcaaaatgaggccaagggcatcatggacgggcgccagctggctgtcccgttcagcctgctgcgggagaacagcctctactggaactactacatcgacagctacctcaagggccagagcccggtggccttcgatctgctgcactggaacagcgacagcaccaatgtggcgggcaagacccacaacagcctgctgcgccgtctctacctggagaaccagctggtgaagggggagctcaagatccgcaacacccgcatcgatctcggcaaggtgaaaaccccggtactgctggtgtcggccgtggacgatcacatcgccctctggcagggcacctggcagggcatgaagctgtttggcggggagcagcgcttcctcctggcggagtccggccacatcgccggcatcatcaacccgccggccgccaacaagtacggcttctggcacaacggggccgaggccgagagcccggagagctggctggcaggggcgacgcaccagggcggctcctggtggcccgagatgatgggctttatccagaaccgtgacgaagggtcggagcccgtccccgcgcgggtgcccgaggaggggctggcccccgcccccggccactatgtcaaggtgcggctcaaccccgtgtttgcctgcccaacagaggaggacgccgcatgacctgccggcctggttcaaccagtcggcagccgactagtggttagccttgcgccttgcttcgctgacgaagaacctctgcgcgctcggcctggccgccgtgctcgcgctggcgggcacggcgcaggcagcgccggcgaccgagctgtcgaccggcccggttaacaccgggccagccggcggcgaaggcctgggcatcaaccaggccattcgcgacggcgaagcccggcgcggcggcacctcgctttccactggcgcgccaaaacccctggcgccgcggccggaatatgcgtcgctgccggtctacgtcggcaaggtcggcgaccagccggtgcggctgcgcctgggccccaagcctgacgagcgcgacagcgtgcgtggcgaatacgccggccgtggcgccggtgtgcgcctgctggcaggcgagtgggaggacggcgccttcctgatggaggagtccgacgacggcacccgcgtatcgggcaactgggaaggcagcatcgacgccagcggcgccgtgcgcggcacctggaccgaatttaaatccga

SEQ ID NO: 41 - DNA, 1732 bp, synthetic construct
  source 1..1732: mol_type = other DNA
gcgcgaattccacgtgcagagagacaatcaaatcatggcgtcaaaggatagcttcgggaaaacaggtgatttgtggtcatcgatgttcaactggatgagcgggacgatgacggccgcggcacagattcagcaggctaatatgcgggccttcgcccaaagcatggaactggcaaccagcgcctatgccaggatgtggggtcagccggtcgaacaggtcgtgccggccgatcgacgcttcaaggatgaggcctggacggaaaacatggccgccgatttgctcaaacagagctacctgatcaccagtcagtggctaatggaaatcgccgatggttggcaggctatcgatcccgatctgcacgaacggacccgcttctggacacagcaactcgtcgacgccaccagcccggctaacttcgccatgaccaacccggtggtgatgcaagagatagcccgcactggcggcatgaacctgatccagggggcgcagaatctattgaaggatgcccaaagtggccggctaacccaagttcctgaggatgcctttgaggtaggtaaggacctggcgatcacgccgggcaaggtcgtatatcgcaaccgcctgattgagttgatccagtacacgccggccacagagacggtccatgaaatccccatcttggtcgtgccgccatggatcaataagtactacgtgatggacatgcagccggagaattcgctgttcaagtacctggtggatgccggcttcaccctgttcaccatcagctggaaaaaccctgatgaaacagttcttgacctggaatgggacgactatctggatctgggcacgctggaagcgctgcgaatggtcaaggaaatcatgggtgtcgagcaggtgaacctggtcggctactgtctaggcgggatcatctcccaggtaactttggcctatctggcggccactggagacgacgcgcagataaacagcgcgacctatttcaccacccaccaggatttcagcgatgcgggcgagatctcggtcttcatcagccggctggacgtgatgttcctggaatggttgatgaagatcagcggcggctacctggatggccggaacctggcggctaccttcaacatgctgcgggccaatgacctgctatggaattacgtggtccacaattatctcttgggccaggaaccggcgtcctttgatctactctactggaataatgacggcaccagggtaccgggcaaggtgcattcattcctgctgcgcgaattcttcctggataacaaactgaaggagcccgagggtattcaggtgaagggcgtgggcattgacctcggtaaaatcacaacgccaacctatgtggtgacggccgaccgggatcacatcgtgccctggcggggcgcattcttggtgcgccagttgcagagcgggccggtgcgcttcatcttgagcggcggcggacatatcgccggggtcattagcccacccactaagaaccgcggcttttggatcaacgaagaagagaaggatgatgctgatgcctggctggccggagcgaccaagcatgacggtagttggtgggtagattggattccatggctcgaggagcgctcgggaagaagggtgaagccaccgacggccgccggcagcgacgagttcaaacccctcatggacgcgccaggcacgtacgttttggagaagtagcctgccggcctggttcaaccagtcggcagccgactagtgcgc

SEQ ID NO: 42 - DNA, 2692 bp, synthetic construct
  source 1..2692: mol_type = other DNA
atccatttaaatcaggcacttgaagcacgcgacggcaagcggcttgcggccatcctgcgccagcacctcctggacaagcgcgacgcggtgctgctgatccaggcaggcgatgccgttggcacgccccaggcataggacgctggcgccaccctcaccccaagaatccgaatagccccatcagcattctttgccccgctgtcaccacggtgacaaccccggttcttactctgcgagcgcattgcggcaaacgcaatccgccatgcggcacctgccgcagcgcacaacaacgcagatgaacaggggaatcaaagatggcagggaaccttgcaccggacaggctggcggggatgtcgcgcggccgtcaattgtgcttctggcgtcaggcagccatcggaagctgtggtatggctgtgcaggtcgtaaatcactgcataattcgtgtcgctcaaggcgcactcccgttctggataatgttttttgcgccgacatcataacggttctggcaaatattctgaaatgagctgttgacaattaatcatcgaactagttaactagtacgcaagttcacagcggataacaatttcacacaggaaacaattgcacgtgcagagagacaatcaaatcatggcgtcaaaggatagcttcgggaaaacaggtgatttgtggtcatcgatgttcaactggatgagcgggacgatgacggccgcggcacagattcagcaggctaatatgcgggccttcgcccaaagcatggaactggcaaccagcgcctatgccaggatgtggggtcagccggtcgaacaggtcgtgccggccgatcgacgcttcaaggatgaggcctggacggaaaacatggccgccgatttgctcaaacagagctacctgatcaccagtcagtggctaatggaaatcgccgatggttggcaggctatcgatcccgatctgcacgaacggacccgcttctggacacagcaactcgtcgacgccaccagcccggctaacttcgccatgaccaacccggtggtgatgcaagagatagcccgcactggcggcatgaacctgatccagggggcgcagaatctattgaaggatgcccaaagtggccggctaacccaagttcctgaggatgcctttgaggtaggtaaggacctggcgatcacgccgggcaaggtcgtatatcgcaaccgcctgattgagttgatccagtacacgccggccacagagacggtccatgaaatccccatcttggtcgtgccgccatggatcaataagtactacgtgatggacatgcagccggagaattcgctgttcaagtacctggtggatgccggcttcaccctgttcaccatcagctggaaaaaccctgatgaaacagttcttgacctggaatgggacgactatctggatctgggcacgctggaagcgctgcgaatggtcaaggaaatcatgggtgtcgagcaggtgaacctggtcggctactgtctaggcgggatcatctcccaggtaactttggcctatctggcggccactggagacgacgcgcagataaacagcgcgacctatttcaccacccaccaggatttcagcgatgcgggcgagatctcggtcttcatcagccggctggacgtgatgttcctggaatggttgatgaagatcagcggcggctacctggatggccggaacctggcggctaccttcaacatgctgcgggccaatgacctgctatggaattacgtggtccacaattatctcttgggccaggaaccggcgtcctttgatctactctactggaataatgacggcaccagggtaccgggcaaggtgcattcattcctgctgcgcgaattcttcctggataacaaactgaaggagcccgagggtattcaggtgaagggcgtgggcattgacctcggtaaaatcacaacgccaacctatgtggtgacggccgaccgggatcacatcgtgccctggcggggcgcattcttggtgcgccagttgcagagcgggccggtgcgcttcatcttgagcggcggcggacatatcgccggggtcattagcccacccactaagaaccgcggcttttggatcaacgaagaagagaaggatgatgctgatgcctggctggccggagcgaccaagcatgacggtagttggtgggtagattggattccatggctcgaggagcgctcgggaagaagggtgaagccaccgacggccgccggcagcgacgagttcaaacccctcatggacgcgccaggcacgtacgttttggagaagtagcctgccggcctggttcaaccagtcggcagccggaattgatcgatactagtatccggccggagcccgtttcgtcacggaacgggttcctcaccgacccttcccccccgcccgatcccctgcaggagattgacaccatgactttccgaccttccaccctggcgcggccgcactggctcgccgccgtgctgatgtgcgcagcgctcgccgcctgcggcggcgactccggcgacagccccaccggctcgcccaacgcggcaccgatcacgccgggtgccccgggtaccggcggcaaccccggccaggggaatggcagcgaccagcctggcgagacgcccgccgtgaagccgcagctgcgctgcgcaccctgaagccgggcctggcccgtctcccctccagaaacatttaaatccga

SEQ ID NO: 43 - DNA, 1732 bp, synthetic construct
  source 1..1732: mol_type = other DNA
gcgccaattgcacgtgcagagagacaatcaaatcatggcgtcaaaggatagcttcgggaaaacaggtgatttgtggtcatcgatgttcaactggatgagcgggacgatgacggccgcggcacagattcagcaggctaatatgcgggccttcgcccaaagcatggaactggcaaccagcgcctatgccaggatgtggggtcagccggtcgaacaggtcgtgccggccgatcgacgcttcaaggatgaggcctggacggaaaacatggccgccgatttgctcaaacagagctacctgatcaccagtcagtggctaatggaaatcgccgatggttggcaggctatcgatcccgatctgcacgaacggacccgcttctggacacagcaactcgtcgacgccaccagcccggctaacttcgccatgaccaacccggtggtgatgcaagagatagcccgcactggcggcatgaacctgatccagggggcgcagaatctattgaaggatgcccaaagtggccggctaacccaagttcctgaggatgcctttgaggtaggtaaggacctggcgatcacgccgggcaaggtcgtatatcgcaaccgcctgattgagttgatccagtacacgccggccacagagacggtccatgaaatccccatcttggtcgtgccgccatggatcaataagtactacgtgatggacatgcagccggagaattcgctgttcaagtacctggtggatgccggcttcaccctgttcaccatcagctggaaaaaccctgatgaaacagttcttgacctggaatgggacgactatctggatctgggcacgctggaagcgctgcgaatggtcaaggaaatcatgggtgtcgagcaggtgaacctggtcggctactgtctaggcgggatcatctcccaggtaactttggcctatctggcggccactggagacgacgcgcagataaacagcgcgacctatttcaccacccaccaggatttcagcgatgcgggcgagatctcggtcttcatcagccggctggacgtgatgttcctggaatggttgatgaagatcagcggcggctacctggatggccggaacctggcggctaccttcaacatgctgcgggccaatgacctgctatggaattacgtggtccacaattatctcttgggccaggaaccggcgtcctttgatctactctactggaataatgacggcaccagggtaccgggcaaggtgcattcattcctgctgcgcgaattcttcctggataacaaactgaaggagcccgagggtattcaggtgaagggcgtgggcattgacctcggtaaaatcacaacgccaacctatgtggtgacggccgaccgggatcacatcgtgccctggcggggcgcattcttggtgcgccagttgcagagcgggccggtgcgcttcatcttgagcggcggcggacatatcgccggggtcattagcccacccactaagaaccgcggcttttggatcaacgaagaagagaaggatgatgctgatgcctggctggccggagcgaccaagcatgacggtagttggtgggtagattggattccatggctcgaggagcgctcgggaagaagggtgaagccaccgacggccgccggcagcgacgagttcaaacccctcatggacgcgccaggcacgtacgttttggagaagtagcctgccggcctggttcaaccagtcggcagccgactagtgcgc

SEQ ID NO: 44 - protein, 551 aa, unidentified; identical to SEQ ID NO: 9

SEQ ID NO: 45 - DNA, 1744 bp, synthetic construct
  source 1..1744: mol_type = other DNA
gcgccaattgcacgtgcagagagacaatcaaatcatggcgtcaaaggatagcttcgggaaaacaggtgatttgtggtcatcgatgttcaactggatgagcgggacgatgacggccgcggcacagattcagcaggctaatatgcgggccttcgcccaaagcatggaactggcaaccagcgcctatgccaggatgtggggtcagccggtcgaacaggtcgtgccggccgatcgacgcttcaaggatgaggcctggacggaaaacatggccgccgatttgctcaaacagagctacctgatcaccagtcagtggctaatggaaatcgccgatggttggcaggctatcgatcccgatctgcacgaacggacccgcttctggacacagcaactcgtcgacgccaccagcccggctaacttcgccatgaccaacccggtggtgatgcaagagatagcccgcactggcggcatgaacctgatccagggggcgcagaatctattgaaggatgcccaaagtggccggctaacccaagttcctgaggatgcctttgaggtaggtaaggacctggcgatcacgccgggcaaggtcgtatatcgcaaccgcctgattgagttgatccagtacacgccggccacagagacggtccatgaaatccccatcttggtcgtgccgccatggatcaataagtactacgtgatggacatgcagccggagaattcgctgttcaagtacctggtggatgccggcttcaccctgttcaccatcagctggaaaaaccctgatgaaacagttcttgacctggaatgggacgactatctggatctgggcacgctggaagcgctgcgaatggtcaaggaaatcatgggtgtcgagcaggtgaacctggtcggctactgtctaggcgggatcatctcccaggtaactttggcctatctggcggccactggagacgacgcgcagataaacagcgcgacctatttcaccacccaccaggatttcagcgatgcgggcgagatctcggtcttcatcagccggctggacgtgatgttcctggaatggttgatgaagatcagcggcggctacctggatggccggaacctggcggctcctttcaacatgctgcgggccaatgacctgctatggaattacgtggtccacaattatctcttgggccaggaaccggcgtcctttgatctactctactggaataatgacggcaccagggtaccgggcaaggtgcattcattcctgctgcgcgaattcttcctggataacaaactgaaggagcccgagggtattcaggtgaagggcgtgggcattgacctcggtaaaatcacaacgccaacctatgtggtgacggccgaccgggatcacatcgtgccctggcggggcgcattcttggtgcgccagttgcagagcgggccggtgcgcttcatcttgagcggcggcggacatatcgccggggtcattagcccacccactaagaaccgcggcttttggatcaacgaagaagagaaggatgatgctgatgcctggctggccggagcgaccaagcatgacggtagttggtgggtagattggattccatggctcgaggagcgctcgggaagaagggtgaagccaccgacggccgccggcagcgacgagttcaaacccctcatggacgcgccaggcacgtacgttttggagaagtagcctgccggcctggttcaaccagtcggcagccggaattgatcgatactagtgcgc

SEQ ID NO: 46 - DNA, 2793 bp, synthetic construct; identical to SEQ ID NO: 34
  source 1..2793: mol_type = other DNA

SEQ ID NO: 47 - DNA, 2858 bp, synthetic construct
  source 1..2858: mol_type = other DNA
atccatttaaatggagttccagaccctgctcgactttatcgccgaagccgaactggaccgcgtcggctgcttcgcctactcgccggtggagggcgccaccgccaatgacctgccgggcgcgctgcccgacgaggtgcgcgaggaacgccgcgcccgcttcatggaagtggccgaagaggtctcggcgcgccgcctgcagcgcaaggtcggccagaccctgcgcgtgctggtggacgaggtcaaccaggatggcggcatcggccgttcgtccgcggatgcgccggaaatcgacggcctcgtctatatcgcgccgccggaacgccacgcccagcgctatcgcgccggcgagttcgtcgacgtgaagatcaccggcgccgatggccacgacctgtggggcgcggtctgaaacgggttgattaggtaaaagtacgctcgttcgatttcgtccgcgtcccgctatactgtgcggtgcaacataacctcatggagacaaagtccaattgcacgtgcagagagacaatcaaatcatgagccaaccatcttatggcccgctgttcgaggccctggcccactacaatgacaagctgctggccatggccaaggcccagacagagcgcaccgcccaggcgctgctgcagaccaatctggacgatctgggccaggtgctggagcagggcagccagcaaccctggcaactgatccaggcccagatgaactggtggcaggatcagctcaagctgatgcagcacaccctgctcaaaagcgcaggccagccgagcgagccggtgatcaccccggagcgcagcgatcgccgcttcaaggccgaggcctggagcgaacaacccatctatgactacctcaagcagtcctacctgctcaccgccaggcacctgctggcctcggtggatgccctggagggcgtcccccagaagagccgggagcggctgcgtttcttcacccgccagtacgtcagcgccatggcccccagcaacttcctggccaccaaccccgagctgctcaagctgaccctggagtccggcggccagaacctggtgcgcgggctggccctcttggccgaggatctggagcgcagcgccgatcagctcaacatccgcctgaccgacgaatccgccttcgagctcgggcgggatctggcgctcaccccgggccgggtggtgcagcgcaccgagctctatgagctgatccagtacagcccgactaccgagacggtgggcaagacacctgtgctgatagtgccccccttcatcaacaagtactacatcatggacatgcggccccagaactccctggtcgcctggctggtcgcccagggccagacggtgttcatgatctcctggcgcaacccgggcgtggcccaggcccaaatcgatctcgacgactacgtggtggacggggtcatcgccgccctggacggggtggaggcggccaccggcgagcgggaggtgcacggcatcggctactgcatcggcggcactgcactgtcgctcgccatgggctggctggcggcgcggcgccagaagcagcgagtgcgcaccgccaccctgttcactaccctgctggacttctcccagccaggggagctcggcatcttcatccacgagcccatcatagcggcgctcgaggcgcaaaatgaggccaagggcatcatggacgggcgccagctggctgtctgcttcagcctgctgcgggagaacagcctctactggaactactacatcgacagctacctcaagggccagagcccggtggccttcgatctgctgcactggaacagcgacagcaccaatgtggcgggcaagacccacaacagcctgctgcgccgtctctacctggagaaccagctggtgaagggggagctcaagatccgcaacacccgcatcgatctcggcaaggtgaaaaccccggtactgctggtgtcggccgtggacgatcacatcgccctctggcagggcacctggcagggcatgaagctgtttggcggggagcagcgcttcctcctggcggagtccggccacatcgccggcatcatcaacccgccggccgccaacaagtacggcttctggcacaacggggccgaggccgagagcccggagagctggctggcaggggcgacgcaccagggcggctcctggtggcccgagatgatgggctttatccagaaccgtgacgaagggtcggagcccgtccccgcgcgggtgcccgaggaggggctggcccccgcccccggccactatgtcaaggtgcggctcaaccccgtgtttgcctgcccaacagaggaggacgccgcatgacctgccggcctggttcaaccagtcggcagccgactagtggttagccttgcgccttgcttcgctgacgaagaacctctgcgcgctcggcctggccgccgtgctcgcgctggcgggcacggcgcaggcagcgccggcgaccgagctgtcgaccggcccggttaacaccgggccagccggcggcgaaggcctgggcatcaaccaggccattcgcgacggcgaagcccggcgcggcggcacctcgctttccactggcgcgccaaaacccctggcgccgcggccggaatatgcgtcgctgccggtctacgtcggcaaggtcggcgaccagccggtgcggctgcgcctgggccccaagcctgacgagcgcgacagcgtgcgtggcgaatacgccggccgtggcgccggtgtgcgcctgctggcaggcgagtgggaggacggcgccttcctgatggaggagtccgacgacggcacccgcgtatcgggcaactgggaaggcagcatcgacgccagcggcgccgtgcgcggcacctggaccgaatttaaatccga

SEQ ID NO: 48 - DNA, 2858 bp, synthetic construct
  source 1..2858: mol_type = other DNA
atccatttaaatggagttccagaccctgctcgactttatcgccgaagccgaactggaccgcgtcggctgcttcgcctactcgccggtggagggcgccaccgccaatgacctgccgggcgcgctgcccgacgaggtgcgcgaggaacgccgcgcccgcttcatggaagtggccgaagaggtctcggcgcgccgcctgcagcgcaaggtcggccagaccctgcgcgtgctggtggacgaggtcaaccaggatggcggcatcggccgttcgtccgcggatgcgccggaaatcgacggcctcgtctatatcgcgccgccggaacgccacgcccagcgctatcgcgccggcgagttcgtcgacgtgaagatcaccggcgccgatggccacgacctgtggggcgcggtctgaaacgggttgattaggtaaaagtacgctcgttcgatttcgtccgcgtcccgctatactgtgcggtgcaacataacctcatggagacaaagtccaattgcacgtgcagagagacaatcaaatcatgagccaaccatcttatggcccgctgttcgaggccctggcccactacaatgacaagctgctggccatggccaaggcccagacagagcgcaccgcccaggcgctgctgcagaccaatctggacgatctgggccaggtgctggagcagggcagccagcaaccctggcaactgatccaggcccagatgaactggtggcaggatcagctcaagctgatgcagcacaccctgctcaaaagcgcaggccagccgagcgagccggtgatcaccccggagcgcagcgatcgccgcttcaaggccgaggcctggagcgaacaacccatctatgactacctcaagcagtcctacctgctcaccgccaggcacctgctggcctcggtggatgccctggagggcgtcccccagaagagccgggagcggctgcgtttcttcacccgccagtacgtcagcgccatggcccccagcaacttcctggccaccaaccccgagctgctcaagctgaccctggagtccggcggccagaacctggtgcgcgggctggccctcttggccgaggatctggagcgcagcgccgatcagctcaacatccgcctgaccgacgaatccgccttcgagctcgggcgggatctggcgctcaccccgggccgggtggtgcagcgcaccgagctctatgagctgatccagtacagcccgactaccgagacggtgggcaagacacctgtgctgatagtgccccccttcatcaacaagtactacatcatggacatgcggccccagaactccctggtcgcctggctggtcgcccagggccagacggtgttcatgatctcctggcgcaacccgggcgtggcccaggcccaaatcgatctcgacgactacgtggtggacggggtcatcgccgccctggacggggtggaggcggccaccggcgagcgggaggtgcacggcatcggctactgcatcggcggcactgcactgtcgctcgccatgggctggctggcggcgcggcgccagaagcagcgagtgcgcaccgccaccctgttcactaccctgctggacttctcccagccaggggagctcggcatcttcatccacgagcccatcatagcggcgctcgaggcgcaaaatgaggccaagggcatcatggacgggcgccagctggctgtcatcttcagcctgctgcgggagaacagcctctactggaactactacatcgacagctacctcaagggccagagcccggtggccttcgatctgctgcactggaacagcgacagcaccaatgtggcgggcaagacccacaacagcctgctgcgccgtctctacctggagaaccagctggtgaagggggagctcaagatccgcaacacccgcatcgatctcggcaaggtgaaaaccccggtactgctggtgtcggccgtggacgatcacatcgccctctggcagggcacctggcagggcatgaagctgtttggcggggagcagcgcttcctcctggcggagtccggccacatcgccggcatcatcaacccgccggccgccaacaagtacggcttctggcacaacggggccgaggccgagagcccggagagctggctggcaggggcgacgcaccagggcggctcctggtggcccgagatgatgggctttatccagaaccgtgacgaagggtcggagcccgtccccgcgcgggtgcccgaggaggggctggcccccgcccccggccactatgtcaaggtgcggctcaaccccgtgtttgcctgcccaacagaggaggacgccgcatgacctgccggcctggttcaaccagtcggcagccgactagtggttagccttgcgccttgcttcgctgacgaagaacctctgcgcgctcggcctggccgccgtgctcgcgctggcgggcacggcgcaggcagcgccggcgaccgagctgtcgaccggcccggttaacaccgggccagccggcggcgaaggcctgggcatcaaccaggccattcgcgacggcgaagcccggcgcggcggcacctcgctttccactggcgcgccaaaacccctggcgccgcggccggaatatgcgtcgctgccggtctacgtcggcaaggtcggcgaccagccggtgcggctgcgcctgggccccaagcctgacgagcgcgacagcgtgcgtggcgaatacgccggccgtggcgccggtgtgcgcctgctggcaggcgagtgggaggacggcgccttcctgatggaggagtccgacgacggcacccgcgtatcgggcaactgggaaggcagcatcgacgccagcggcgccgtgcgcggcacctggaccgaatttaaatccga

SEQ ID NO: 49 - DNA, 2858 bp, synthetic construct
  source 1..2858: mol_type = other DNA
atccatttaaatggagttccagaccctgctcgactttatcgccgaagccgaactggaccgcgtcggctgcttcgcctactcgccggtggagggcgccaccgccaatgacctgccgggcgcgctgcccgacgaggtgcgcgaggaacgccgcgcccgcttcatggaagtggccgaagaggtctcggcgcgccgcctgcagcgcaaggtcggccagaccctgcgcgtgctggtggacgaggtcaaccaggatggcggcatcggccgttcgtccgcggatgcgccggaaatcgacggcctcgtctatatcgcgccgccggaacgccacgcccagcgctatcgcgccggcgagttcgtcgacgtgaagatcaccggcgccgatggccacgacctgtggggcgcggtctgaaacgggttgattaggtaaaagtacgctcgttcgatttcgtccgcgtcccgctatactgtgcggtgcaacataacctcatggagacaaagtccaattgcacgtgcagagagacaatcaaatcatgagccaaccatcttatggcccgctgttcgaggccctggcccactacaatgacaagctgctggccatggccaaggcccagacagagcgcaccgcccaggcgctgctgcagaccaatctggacgatctgggccaggtgctggagcagggcagccagcaaccctggcaactgatccaggcccagatgaactggtggcaggatcagctcaagctgatgcagcacaccctgctcaaaagcgcaggccagccgagcgagccggtgatcaccccggagcgcagcgatcgccgcttcaaggccgaggcctggagcgaacaacccatctatgactacctcaagcagtcctacctgctcaccgccaggcacctgctggcctcggtggatgccctggagggcgtcccccagaagagccgggagcggctgcgtttcttcacccgccagtacgtcagcgccatggcccccagcaacttcctggccaccaaccccgagctgctcaagctgaccctggagtccggcggccagaacctggtgcgcgggctggccctcttggccgaggatctggagcgcagcgccgatcagctcaacatccgcctgaccgacgaatccgccttcgagctcgggcgggatctggcgctcaccccgggccgggtggtgcagcgcaccgagctctatgagctgatccagtacagcccgactaccgagacggtgggcaagacacctgtgctgatagtgccccccttcatcaacaagtactacatcatggacatgcggccccagaactccctggtcgcctggctggtcgcccagggccagacggtgttcatgatctcctggcgcaacccgggcgtggcccaggcccaaatcgatctcgacgactacgtggtggacggggtcatcgccgccctggacggggtggaggcggccaccggcgagcgggaggtgcacggcatcggctactgcatcggcggcactgcactgtcgctcgccatgggctggctggcggcgcggcgccagaagcagcgagtgcgcaccgccaccctgttcactaccctgctggacttctcccagccaggggagctcggcatcttcatccacgagcccatcatagcggcgctcgaggcgcaaaatgaggccaagggcatcatggacgggcgccagctggctgtcgtgttcagcctgctgcgggagaacagcctctactggaactactacatcgacagctacctcaagggccagagcccggtggccttcgatctgctgcactggaacagcgacagcaccaatgtggcgggcaagacccacaacagcctgctgcgccgtctctacctggagaaccagctggtgaagggggagctcaagatccgcaacacccgcatcgatctcggcaaggtgaaaaccccggtactgctggtgtcggccgtggacgatcacatcgccctctggcagggcacctggcagggcatgaagctgtttggcggggagcagcgcttcctcctggcggagtccggccacatcgccggcatcatcaacccgccggccgccaacaagtacggcttctggcacaacggggccgaggccgagagcccggagagctggctggcaggggcgacgcaccagggcggctcctggtggcccgagatgatgggctttatccagaaccgtgacgaagggtcggagcccgtccccgcgcgggtgcccgaggaggggctggcccccgcccccggccactatgtcaaggtgcggctcaaccccgtgtttgcctgcccaacagaggaggacgccgcatgacctgccggcctggttcaaccagtcggcagccgactagtggttagccttgcgccttgcttcgctgacgaagaacctctgcgcgctcggcctggccgccgtgctcgcgctggcgggcacggcgcaggcagcgccggcgaccgagctgtcgaccggcccggttaacaccgggccagccggcggcgaaggcctgggcatcaaccaggccattcgcgacggcgaagcccggcgcggcggcacctcgctttccactggcgcgccaaaacccctggcgccgcggccggaatatgcgtcgctgccggtctacgtcggcaaggtcggcgaccagccggtgcggctgcgcctgggccccaagcctgacgagcgcgacagcgtgcgtggcgaatacgccggccgtggcgccggtgtgcgcctgctggcaggcgagtgggaggacggcgccttcctgatggaggagtccgacgacggcacccgcgtatcgggcaactgggaaggcagcatcgacgccagcggcgccgtgcgcggcacctggaccgaatttaaatccga

SEQ ID NO: 50 - DNA, 2858 bp, synthetic construct
  source 1..2858: mol_type = other DNA
atccatttaaatggagttccagaccctgctcgactttatcgccgaagccgaactggaccgcgtcggctgcttcgcctactcgccggtggagggcgccaccgccaatgacctgccgggcgcgctgcccgacgaggtgcgcgaggaacgccgcgcccgcttcatggaagtggccgaagaggtctcggcgcgccgcctgcagcgcaaggtcggccagaccctgcgcgtgctggtggacgaggtcaaccaggatggcggcatcggccgttcgtccgcggatgcgccggaaatcgacggcctcgtctatatcgcgccgccggaacgccacgcccagcgctatcgcgccggcgagttcgtcgacgtgaagatcaccggcgccgatggccacgacctgtggggcgcggtctgaaacgggttgattaggtaaaagtacgctcgttcgatttcgtccgcgtcccgctatactgtgcggtgcaacataacctcatggagacaaagtccaattgcacgtgcagagagacaatcaaatcatgagccaaccatcttatggcccgctgttcgaggccctggcccactacaatgacaagctgctggccatggccaaggcccagacagagcgcaccgcccaggcgctgctgcagaccaatctggacgatctgggccaggtgctggagcagggcagccagcaaccctggcaactgatccaggcccagatgaactggtggcaggatcagctcaagctgatgcagcacaccctgctcaaaagcgcaggccagccgagcgagccggtgatcaccccggagcgcagcgatcgccgcttcaaggccgaggcctggagcgaacaacccatctatgactacctcaagcagtcctacctgctcaccgccaggcacctgctggcctcggtggatgccctggagggcgtcccccagaagagccgggagcggctgcgtttcttcacccgccagtacgtcagcgccatggcccccagcaacttcctggccaccaaccccgagctgctcaagctgaccctggagtccggcggccagaacctggtgcgcgggctggccctcttggccgaggatctggagcgcagcgccgatcagctcaacatccgcctgaccgacgaatccgccttcgagctcgggcgggatctggcgctcaccccgggccgggtggtgcagcgcaccgagctctatgagctgatccagtacagcccgactaccgagacggtgggcaagacacctgtgctgatagtgccccccttcatcaacaagtactacatcatggacatgcggccccagaactccctggtcgcctggctggtcgcccagggccagacggtgttcatgatctcctggcgcaacccgggcgtggcccaggcccaaatcgatctcgacgactacgtggtggacggggtcatcgccgccctggacggggtggaggcggccaccggcgagcgggaggtgcacggcatcggctactgcatcggcggcactgcactgtcgctcgccatgggctggctggcggcgcggcgccagaagcagcgagtgcgcaccgccaccctgttcactaccctgctggacttctcccagccaggggagctcggcatcttcatccacgagcccatcatagcggcgctcgaggcgcaaaatgaggccaagggcatcatggacgggcgccagctggctgtcaccttcagcctgctgcgggagaacagcctctactggaactactacatcgacagctacctcaagggccagagcccggtggccttcgatctgctgcactggaacagcgacagcaccaatgtggcgggcaagacccacaacagcctgctgcgccgtctctacctggagaaccagctggtgaagggggagctcaagatccgcaacacccgcatcgatctcggcaaggtgaaaaccccggtactgctggtgtcggccgtggacgatcacatcgccctctggcagggcacctggcagggcatgaagctgtttggcggggagcagcgcttcctcctggcggagtccggccacatcgccggcatcatcaacccgccggccgccaacaagtacggcttctggcacaacggggccgaggccgagagcccggagagctggctggcaggggcgacgcaccagggcggctcctggtggcccgagatgatgggctttatccagaaccgtgacgaagggtcggagcccgtccccgcgcgggtgcccgaggaggggctggcccccgcccccggccactatgtcaaggtgcggctcaaccccgtgtttgcctgcccaacagaggaggacgccgcatgacctgccggcctggttcaaccagtcggcagccgactagtggttagccttgcgccttgcttcgctgacgaagaacctctgcgcgctcggcctggccgccgtgctcgcgctggcgggcacggcgcaggcagcgccggcgaccgagctgtcgaccggcccggttaacaccgggccagccggcggcgaaggcctgggcatcaaccaggccattcgcgacggcgaagcccggcgcggcggcacctcgctttccactggcgcgccaaaacccctggcgccgcggccggaatatgcgtcgctgccggtctacgtcggcaaggtcggcgaccagccggtgcggctgcgcctgggccccaagcctgacgagcgcgacagcgtgcgtggcgaatacgccggccgtggcgccggtgtgcgcctgctggcaggcgagtgggaggacggcgccttcctgatggaggagtccgacgacggcacccgcgtatcgggcaactgggaaggcagcatcgacgccagcggcgccgtgcgcggcacctggaccgaatttaaatccga

SEQ ID NO: 51 - DNA, 2858 bp, synthetic construct; identical to SEQ ID NO: 49
  source 1..2858: mol_type = other DNA

SEQ ID NO: 52 - DNA, 2858 bp, synthetic construct; identical to SEQ ID NO: 49
  source 1..2858: mol_type = other DNA